European Patent Application EP 4 674 959 A1, published January 7, 2026. Title: ニッキング酵素、ＤＮＡ編集システム、標的ＤＮＡの編集方法、及び標的ＤＮＡが編集された細胞の製造方法. Applicant: SUMITOMO CHEMICAL COMPANY, LIMITED. The sequence listing filed with the application follows.

SEQUENCE LISTING (370 sequences)

SEQ ID NO: 1 - DNA, 21 bp, synthetic construct
  misc_feature 1..21: note = FokI_FW
  source 1..21: mol_type = other DNA
cacagagtggccctgaagcag

SEQ ID NO: 2 - DNA, 21 bp, synthetic construct
  misc_feature 1..21: note = FokI_RV
  source 1..21: mol_type = other DNA
gccactgtgctggattaaaag

SEQ ID NO: 3 - DNA, 43 bp, synthetic construct
  misc_feature 1..43: note = TALE63-RinfFokI
  source 1..43: mol_type = other DNA
cagggccactctgtgtgatgtcctctcggggatccttctgttg

SEQ ID NO: 4 - DNA, 42 bp, synthetic construct
  misc_feature 1..42: note = Vector-FinfFokI
  source 1..42: mol_type = other DNA
atccagcacagtggcgaattctgcagatatccagcacagtgg

SEQ ID NO: 5 - DNA, 45 bp, synthetic construct
  misc_feature 1..45: note = ND1F_inf63-2
  source 1..45: mol_type = other DNA
cgagtggcaggttcccttgttaagggcgaaatggagaaaaagaag

SEQ ID NO: 6 - DNA, 48 bp, synthetic construct
  misc_feature 1..48: note = ND1R_inf63
  source 1..48: mol_type = other DNA
atatctgcagaattcttagaagatgatctcgtcattgttgaacttatc

SEQ ID NO: 7 - DNA, 42 bp, synthetic construct
  misc_feature 1..42: note = ND2F_inf63
  source 1..42: mol_type = other DNA
cgagtggcaggttccattgttaagagcagcattgagatgagc

SEQ ID NO: 8 - DNA, 46 bp, synthetic construct
  misc_feature 1..46: note = ND2R_inf63
  source 1..46: mol_type = other DNA
atatctgcagaattcttagaactgaatctccttattcaggaaagag

SEQ ID NO: 9 - DNA, 48 bp, synthetic construct
  misc_feature 1..48: note = ND1monoR_inf63
  source 1..48: mol_type = other DNA
atatctgcagaattcttaaaagataatctcatcgttgttgaatttatc

SEQ ID NO: 10 - DNA, 49 bp, synthetic construct
  misc_feature 1..49: note = ND2monoR_inf63
  source 1..49: mol_type = other DNA
atatctgcagaattcttagaactggatctctttgttcagaaacgaattc

SEQ ID NO: 11 - DNA, 26 bp, synthetic construct
  misc_feature 1..26: note = TALE_63_R
  source 1..26: mol_type = other DNA
ggaacctgccactcgatgtgatgtcc

SEQ ID NO: 12 - DNA, 27 bp, synthetic construct
  misc_feature 1..27: note = TALEvector_F
  source 1..27: mol_type = other DNA
gaattctgcagatatccagcacagtgg

SEQ ID NO: 13 - DNA, 24 bp, synthetic construct
  misc_feature 1..24: note = TALE_47_R
  source 1..24: mol_type = other DNA
ggatctgatcaattccggcgcgtg

SEQ ID NO: 14 - DNA, 39 bp, synthetic construct
  misc_feature 1..39: note = EGFP_F+bam
  source 1..39: mol_type = other DNA
taccgagctcggatcatggtgagcaagggcgaggagctg

SEQ ID NO: 15 - DNA, 21 bp, synthetic construct
  misc_feature 1..21: note = EGFP_600R
  source 1..21: mol_type = other DNA
gtggttgtcgggcagcagcac

SEQ ID NO: 16 - DNA, 36 bp, synthetic construct
  misc_feature 1..36: note = EGFP_600R+linker
  source 1..36: mol_type = other DNA
gctagcggatcctcagtggttgtcgggcagcagcac

SEQ ID NO: 17 - DNA, 24 bp, synthetic construct
  misc_feature 1..24: note = EGFP_120F
  source 1..24: mol_type = other DNA
ggcaagctgaccctgaagttcatc

SEQ ID NO: 18 - DNA, 40 bp, synthetic construct
  misc_feature 1..40: note = EGFP_R+rv
  source 1..40: mol_type = other DNA
gccactgtgctggatttacttgtacagctcgtccatgccg

SEQ ID NO: 19 - DNA, 63 bp, synthetic construct
  misc_feature 1..63: note = linker+EGFP_120F
  source 1..63: mol_type = other DNA
tgaggatccgctagcctgcaggtcgacgaattcgatatcggcaagctgaccctgaagttcatc

SEQ ID NO: 20 - DNA, 27 bp, synthetic construct
  misc_feature 1..27: note = TALE-CR
  source 1..27: mol_type = other DNA
gagacgaccggtggaaagcgggcagtg

SEQ ID NO: 21 - DNA, 24 bp, synthetic construct
  misc_feature 1..24: note = Amp_R
  source 1..24: mol_type = other DNA
cactcatggttatggcagcactgc

SEQ ID NO: 22 - DNA, 30 bp, synthetic construct
  misc_feature 1..30: note = ND1-N_F
  source 1..30: mol_type = other DNA
cttgttaagggcgaaatggagaaaaagaag

SEQ ID NO: 23 - DNA, 29 bp, synthetic construct
  misc_feature 1..29: note = Amp_F
  source 1..29: mol_type = other DNA
ccataaccatgagtgataacactgcggcc

SEQ ID NO: 24 - DNA, 29 bp, synthetic construct
  misc_feature 1..29: note = WT-CF
  source 1..29: mol_type = other DNA
tccaccggtcgtctccacccctgagcagg

SEQ ID NO: 25 - DNA, 42 bp, synthetic construct
  misc_feature 1..42: note = WT-63R_infND1
  source 1..42: mol_type = other DNA
ttcgcccttaacaagtgccactcgatgtgatgtcctctcggg

SEQ ID NO: 26 - DNA, 42 bp, synthetic construct
  misc_feature 1..42: note = WT-75R_infND1
  source 1..42: mol_type = other DNA
ttcgcccttaacaaggaagaatccgagcacgcggaccacttg

SEQ ID NO: 27 - DNA, 41 bp, synthetic construct
  misc_feature 1..41: note = WT-90R_infND1
  source 1..41: mol_type = other DNA
ttcgcccttaacaagagtcatggcgtcatcgaacgcttgtg

SEQ ID NO: 28 - DNA, 44 bp, synthetic construct
  misc_feature 1..44: note = WT-105R_infND1
  source 1..44: mol_type = other DNA
ttcgcccttaacaagtctacgaaagagctgcagcagtccgtgtc

SEQ ID NO: 29 - DNA, 43 bp, synthetic construct
  misc_feature 1..43: note = WT-120_infND1
  source 1..43: mol_type = other DNA
ttcgcccttaacaaggggaggcagtgtgcccgagcgggcctcc

SEQ ID NO: 30 - DNA, 43 bp, synthetic construct
  misc_feature 1..43: note = WT-135R_infND1
  source 1..43: mol_type = other DNA
ttcgcccttaacaagtttcataccgctcgcttggagaatcctg

SEQ ID NO: 31 - DNA, 41 bp, synthetic construct
  misc_feature 1..41: note = WT-150R_infND1
  source 1..41: mol_type = other DNA
ttcgcccttaacaagcgcctggtcaggtgtctgagttgacg

SEQ ID NO: 32 - DNA, 42 bp, synthetic construct
  misc_feature 1..42: note = WT-165R_infND1
  source 1..42: mol_type = other DNA
ttcgcccttaacaagcgcgtccaaatccctctccagcgagtc

SEQ ID NO: 33 - DNA, 42 bp, synthetic construct
  misc_feature 1..42: note = WT-180R_infND1
  source 1..42: mol_type = other DNA
ttcgcccttaacaaggctggctgacgcgcgagtttggtcccc

SEQ ID NO: 34 - DNA, 43 bp, synthetic construct
  misc_feature 1..43: note = TALE-0_R_infND1
  source 1..43: mol_type = other DNA
ttcgcccttaacaagctccagtgcgggtctgcccccgttgttg

SEQ ID NO: 35 - DNA, 43 bp, synthetic construct
  misc_feature 1..43: note = TALE-12_R_infND1
  source 1..43: mol_type = other DNA
ttcgcccttaacaagcgcggggtccggcctcgaaagctgggcc

SEQ ID NO: 36 - DNA, 41 bp, synthetic construct
  misc_feature 1..41: note = TALE-24_R_infND1
  source 1..41: mol_type = other DNA
ttcgcccttaacaagcgctacaagatgatcattagtgagtg

SEQ ID NO: 37 - DNA, 42 bp, synthetic construct
  misc_feature 1..42: note = TALE-36_R_infND1
  source 1..42: mol_type = other DNA
ttcgcccttaacaagcactgcatccatggcaggacgtccgcc

SEQ ID NO: 38 - DNA, 41 bp, synthetic construct
  misc_feature 1..41: note = GSSx4+5'ad._F
  source 1..41: mol_type = other DNA
ccgggtggggtctagtggctccagcggatcaagtggcagct

SEQ ID NO: 39 - DNA, 41 bp, synthetic construct
  misc_feature 1..41: note = GSSx4+5'ad._R
  source 1..41: mol_type = other DNA
ccggagctgccacttgatccgctggagccactagaccccac

SEQ ID NO: 40 - DNA, 41 bp, synthetic construct
  misc_feature 1..41: note = SAGGx3+5'ad._F
  source 1..41: mol_type = other DNA
ccgggtgtctgctggcgggtccgccgggggcagtgctggcg

SEQ ID NO: 41 - DNA, 41 bp, synthetic construct
  misc_feature 1..41: note = SAGGx3+5'ad._R
  source 1..41: mol_type = other DNA
gatccgccagcactgcccccggcggacccgccagcagacac

SEQ ID NO: 42 - DNA, 50 bp, synthetic construct
  misc_feature 1..50: note = GGGGSx3+5'ad._F
  source 1..50: mol_type = other DNA
ccgggtggggggcggagggtctggcggagggggctctggagggggcggat

SEQ ID NO: 43 - DNA, 50 bp, synthetic construct
  misc_feature 1..50: note = GGGGSx3+5'ad._R
  source 1..50: mol_type = other DNA
ccggatccgccccctccagagccccctccgccagaccctccgccccccac

SEQ ID NO: 44 - DNA, 36 bp, synthetic construct
  misc_feature 1..36: note = GSSx4_F
  source 1..36: mol_type = other DNA
ccgggtctagtggctccagcggatcaagtggcagct

SEQ ID NO: 45 - DNA, 36 bp, synthetic construct
  misc_feature 1..36: note = GSSx4_R
  source 1..36: mol_type = other DNA
ccggagctgccacttgatccgctggagccactagac

SEQ ID NO: 46 - DNA, 63 bp, synthetic construct
  misc_feature 1..63: note = GSSx7_F
  source 1..63: mol_type = other DNA
ccgggtctagtggctccagcggatcaagtgggagttctggcagctcaggatctagtggcagct

SEQ ID NO: 47 - DNA, 63 bp, synthetic construct
  misc_feature 1..63: note = GSSx7_R
  source 1..63: mol_type = other DNA
ccggagctgccactagatcctgagctgccagaactcccacttgatccgctggagccactagac

SEQ ID NO: 48 - DNA, 36 bp, synthetic construct
  misc_feature 1..36: note = SAGGx3_F
  source 1..36: mol_type = other DNA
gatctgctggcgggtccgccgggggcagtgctggcg

SEQ ID NO: 49 - DNA, 36 bp, synthetic construct
  misc_feature 1..36: note = SAGGx3_R
  source 1..36: mol_type = other DNA
gatccgccagcactgcccccggcggacccgccagca

SEQ ID NO: 50 - DNA, 48 bp, synthetic construct
  misc_feature 1..48: note = SAGGx4_F
  source 1..48: mol_type = other DNA
gatctgctggcgggtccgccgggggctcagcaggagggagtgctggcg

SEQ ID NO: 51 - DNA, 48 bp, synthetic construct
  misc_feature 1..48: note = SAGGx4_R
  source 1..48: mol_type = other DNA
gatccgccagcactccctcctgctgagcccccggcggacccgccagca

SEQ ID NO: 52 - DNA, 45 bp, synthetic construct
  misc_feature 1..45: note = GGGGSx3_F
  source 1..45: mol_type = other DNA
ccgggggcggagggtctggcggagggggctctggagggggcggat

SEQ ID NO: 53 - DNA, 45 bp, synthetic construct
  misc_feature 1..45: note = GGGGSx3_R
  source 1..45: mol_type = other DNA
ccggatccgccccctccagagccccctccgccagaccctccgccc

SEQ ID NO: 54 - DNA, 60 bp, synthetic construct
  misc_feature 1..60: note = GGGGSx4_F
  source 1..60: mol_type = other DNA
ccgggggcggagggtctggcggagggggctctggagggggcggatcagggggcggagggt

SEQ ID NO: 55 - DNA, 60 bp, synthetic construct
  misc_feature 1..60: note = GGGGSx4_R
  source 1..60: mol_type = other DNA
ccggaccctccgccccctgatccgccccctccagagccccctccgccagaccctccgccc

SEQ ID NO: 56 - DNA, 33 bp, synthetic construct
  misc_feature 1..33: note = bamND1_F
  source 1..33: mol_type = other DNA
ggatccatgaccgcggtcctcgtgaaaggggag

SEQ ID NO: 57 - DNA, 42 bp, synthetic construct
  misc_feature 1..42: note = 95aa_R_inf_bamND1
  source 1..42: mol_type = other DNA
cgcggtcatggatccgctagatccgcttccagatccgctgcc

SEQ ID NO: 58 - DNA, 33 bp, synthetic construct
  misc_feature 1..33: note = mroND1_F
  source 1..33: mol_type = other DNA
tccggaatgaccgcggtcctcgtgaaaggggag

SEQ ID NO: 59 - DNA, 42 bp, synthetic construct
  misc_feature 1..42: note = 95aa_R_inf_mroND1
  source 1..42: mol_type = other DNA
cgcggtcattccggagctagatccgcttccagatccgctgcc

SEQ ID NO: 60 - DNA, 1461 bp, synthetic construct
  misc_feature 1..1461: note = FokI-95-FokI
  source 1..1461: mol_type = other DNA
  CDS 1..1461
cagctggtgaagtctgagctggaggagaagaagagcgagctgcggcacaagctgaagtacgtgccacacgagtatatcgagctgatcgagatcgcccggaactccacccaggacagaatcctggagatgaaagtgatggagttctttatgaaggtgtacggatataggggcaagcacctgggaggctccagaaagcctgatggcgccatctacaccgtgggctctccaatcgactatggcgtgatcgtggatacaaaggcctactccggcggctataatctgcccatcggccaggccgatgagatgcagaggtacgtggaggagaaccagacccgcaataagcacatcaaccccaatgagtggtggaaggtgtatcctagctccgtgacagagttcaagtttctgttcgtgtctggccacttcaagggcaactacaaggcccagctgaccagactgaatcacatcacaaactgtaatggagccgtgctgagcgtggaggagctgctgatcggcggcgagatgatcaaggcaggcaccctgacactggaggaggtgcggagaaagttcaacaatggcgagatcaactttggaagcggatccggatctggaagcatcaccaggaccacaaaccctcgcaatgtggtgccaaagatctacatgtccgccggctctatccctctgaccacacacatcacaaacagcatccagccaaccctgtggacaatcggatccatcaatggagtggcaccactggccaagtctatcaagctgggcatccctgtgaccggcagcgcctacacagaccagaccacagccatggtgcggaagaaggtgagcgtgttcatgggcagcggatctggaagcggatctagccagctggtgaagtccgaactggaagagaagaagtctgagctgcgccataagctgaagtatgtgcctcatgaatacattgaactgattgagatcgccaggaacagcacccaggaccgcatcctggaaatgaaagtgatggagttctttatgaaagtctatggctacagaggcaagcacctgggcggcagcagaaagccagacggagctatctacactgtgggctcccccattgattacggcgtgatcgtcgatacaaaggcctacagtggaggatacaatctgcctattggacaggctgatgagatgcagaggtatgtggaggaaaatcagactagaaataagcacatcaacccaaacgaatggtggaaggtgtacccctcctctgtgacagagtttaagttcctgttcgtgagcggacacttcaagggaaactataaggcccagctgacccggctgaatcatattacaaactgcaatggcgccgtgctgtctgtcgaagaactgctgattggaggagagatgatcaaggccggcaccctgacactggaagaggtgaggcgcaagttcaacaacggagagatcaacttt

SEQ ID NO: 61 - protein, 487 aa, synthetic construct
  REGION 1..487: note = Synthetic Construct
QLVKSELEEKKSELRHKLKYVPHEYIELIEIARNSTQDRILEMKVMEFFMKVYGYRGKHLGGSRKPDGAIYTVGSPIDYGVIVDTKAYSGGYNLPIGQADEMQRYVEENQTRNKHINPNEWWKVYPSSVTEFKFLFVSGHFKGNYKAQLTRLNHITNCNGAVLSVEELLIGGEMIKAGTLTLEEVRRKFNNGEINFGSGSGSGSITRTTNPRNVVPKIYMSAGSIPLTTHITNSIQPTLWTIGSINGVAPLAKSIKLGIPVTGSAYTDQTTAMVRKKVSVFMGSGSGSGSSQLVKSELEEKKSELRHKLKYVPHEYIELIEIARNSTQDRILEMKVMEFFMKVYGYRGKHLGGSRKPDGAIYTVGSPIDYGVIVDTKAYSGGYNLPIGQADEMQRYVEENQTRNKHINPNEWWKVYPSSVTEFKFLFVSGHFKGNYKAQLTRLNHITNCNGAVLSVEELLIGGEMIKAGTLTLEEVRRKFNNGEINF

SEQ ID NO: 62 - DNA, 1356 bp, synthetic construct
  misc_feature 1..1356: note = FokI-60-FokI
  source 1..1356: mol_type = other DNA
  CDS 1..1356
cagctggtgaagtccgagctggaggagaagaagtctgagctgaggcacaagctgaagtacgtgccacacgagtatatcgagctgatcgagatcgccaggaacagcacccaggaccgcatcctggagatgaaagtgatggagttctttatgaaggtgtacggctataggggcaagcacctgggaggcagccgcaagccagatggagccatctacaccgtgggctcccccatcgactatggcgtgatcgtggatacaaaggcctactccggcggctataatctgcccatcggccaggccgatgagatgcagcggtacgtggaggagaaccagaccagaaataagcacatcaaccctaatgagtggtggaaggtgtatccaagctccgtgacagagttcaagtttctgttcgtgagcggccacttcaagggcaactacaaggcccagctgacccggctgaatcacatcacaaactgtaatggagccgtgctgtccgtggaggagctgctgatcggcggcgagatgatcaaggcaggcaccctgacactggaggaggtgcggagaaagttcaacaatggcgagatcaactttggcggcggcggctcaggcggcggcggctctggaggaggaggaagcggaggaggaggaagcgggggcggcggctctggcggcggcggcagcggaggaggaggatctggaggaggaggatccggcggcggcggcagcgggggaggagggagcggaggaggagggtccggaggaggcggcagccagctggtcaaaagcgaactggaggagaagaagtccgagctgagacataagctgaagtatgtgcctcatgaatacattgaactgattgagatcgcccggaactctacccaggacagaatcctggaaatgaaagtgatggagttctttatgaaagtctatggatacagaggcaagcacctgggcggctctcgcaagcctgacggcgctatctacactgtgggcagcccaattgattacggcgtgatcgtcgatacaaaggcctacagtggaggctataatctgccaatcggacaggcagacgagatgcagcggtatgtggaggaaaatcagactaggaataagcacatcaaccccaacgaatggtggaaggtgtacccttctagcgtgacagagtttaagttcctgttcgtgagcggacactttaagggaaattataaagctcagctgactcggctgaatcatattacaaactgcaatggagccgtgctgagtgtcgaagaactgctgattggaggcgagatgatcaaggccggcaccctgacactggaagaggtgaggcgcaagttcaacaacggagagatcaacttt

SEQ ID NO: 63 - protein, 452 aa, synthetic construct
  REGION 1..452: note = Synthetic Construct
QLVKSELEEKKSELRHKLKYVPHEYIELIEIARNSTQDRILEMKVMEFFMKVYGYRGKHLGGSRKPDGAIYTVGSPIDYGVIVDTKAYSGGYNLPIGQADEMQRYVEENQTRNKHINPNEWWKVYPSSVTEFKFLFVSGHFKGNYKAQLTRLNHITNCNGAVLSVEELLIGGEMIKAGTLTLEEVRRKFNNGEINFGGGGSGGGGSGGGGSGGGGSGGGGSGGGGSGGGGSGGGGSGGGGSGGGGSGGGGSGGGGSQLVKSELEEKKSELRHKLKYVPHEYIELIEIARNSTQDRILEMKVMEFFMKVYGYRGKHLGGSRKPDGAIYTVGSPIDYGVIVDTKAYSGGYNLPIGQADEMQRYVEENQTRNKHINPNEWWKVYPSSVTEFKFLFVSGHFKGNYKAQLTRLNHITNCNGAVLSVEELLIGGEMIKAGTLTLEEVRRKFNNGEINF

SEQ ID NO: 64 - DNA, 528 bp, synthetic construct
  misc_feature 1..528: note = N-terminal domain of TALE63
  source 1..528: mol_type = other DNA
  CDS 1..528
atggactataaggaccacgacggagactacaaggatcatgatattgattacaaagacgatgacgataagatggccccaaagaagaagcggaaggtcggtatccacggagtcccagcagccgtagatttgagaactttgggatattcacagcagcagcaggaaaagatcaagcccaaagtgaggtcgacagtcgcgcagcatcacgaagcgctggtgggtcatgggtttacacatgcccacatcgtagccttgtcgcagcaccctgcagcccttggcacggtcgccgtcaagtaccaggacatgattgcggcgttgccggaagccacacatgaggcgatcgtcggtgtggggaaacagtggagcggagcccgagcgcttgaggccctgttgacggtcgcgggagagctgagagggcctccccttcagctggacacgggccagttgctgaagatcgcgaagcggggaggagtcacggcggtcgaggcggtacacgcgtggcgcaatgcgctcacgggagcacccctcaag

SEQ ID NO: 65 - protein, 176 aa, synthetic construct
  REGION 1..176: note = Synthetic Construct
MDYKDHDGDYKDHDIDYKDDDDKMAPKKKRKVGIHGVPAAVDLRTLGYSQQQQEKIKPKVRSTVAQHHEALVGHGFTHAHIVALSQHPAALGTVAVKYQDMIAALPEATHEAIVGVGKQWSGARALEALLTVAGELRGPPLQLDTGQLLKIAKRGGVTAVEAVHAWRNALTGAPLK

SEQ ID NO: 66 - DNA, 252 bp, synthetic construct
  misc_feature 1..252: note = C-terminal domain of TALE63
  source 1..252: mol_type = other DNA
  CDS 1..252
acccctgagcaggtagtggctattgcatccaacaacgggggcagacccgcactggagtcaatcgtggcccagctttcgaggccggaccccgcgctggccgcactcactaatgatcatcttgtagcgctggcctgcctcggcggacgacccgccttggatgcggtgaagaaggggctcccgcacgcgcctgcattgattaagcggaccaacagaaggatccccgagaggacatcacacagagtggccggttcc

SEQ ID NO: 67 - protein, 84 aa, synthetic construct
  REGION 1..84: note = Synthetic Construct
TPEQVVAIASNNGGRPALESIVAQLSRPDPALAALTNDHLVALACLGGRPALDAVKKGLPHAPALIKRTNRRIPERTSHRVAGS

SEQ ID NO: 68 - DNA, 567 bp, synthetic construct
  misc_feature 1..567: note = N-terminal domain of TALE47
  source 1..567: mol_type = other DNA
  CDS 1..567
atggcttcctcccctccaaagaaaaagagaaaggttgcggccgctgactacaaggatgacgacgataaaagttggaaggacgcaagtggttggtctagaatgcatgcggccccgcgacggcgtgctgcgcaaccctccgacgcttcgccggccgcgcaggtggatctacgcacgctcggctacagtcagcagcagcaagagaagatcaaaccgaaggtgcgttcgacagtggcgcagcaccacgaggcactggtgggccatgggtttacacacgcgcacatcgttgcgctcagccaacacccggcagcgttagggaccgtcgctgtcacgtatcagcacataatcacggcgttgccagaggcgacacacgaagacatcgttggcgtcggcaaacagtggtccggcgcacgcgccctggaggccttgctcacggatgcgggggagttgagaggtccgccgttacagttggacacaggccaacttgtgaagattgcaaaacgtggcggcgtgaccgcaatggaggcagtgcatgcatcgcgcaatgcgctcacgggagcacccctcaag

SEQ ID NO: 69 - protein, 189 aa, synthetic construct
  REGION 1..189: note = Synthetic Construct
MASSPPKKKRKVAAADYKDDDDKSWKDASGWSRMHAAPRRRAAQPSDASPAAQVDLRTLGYSQQQQEKIKPKVRSTVAQHHEALVGHGFTHAHIVALSQHPAALGTVAVTYQHIITALPEATHEDIVGVGKQWSGARALEALLTDAGELRGPPLQLDTGQLVKIAKRGGVTAMEAVHASRNALTGAPLK

SEQ ID NO: 70 - DNA, 204 bp, synthetic construct
  misc_feature 1..204: note = C-terminal domain of TALE47
  source 1..204: mol_type = other DNA
  CDS 1..204
acccctgagcaggtagtggctattgcatccaacaacgggggcagacccgcactggagtcaatcgtggcccagctttcgaggccggaccccgcgctggccgcactcactaatgatcatcttgtagcgctggcctgcctcggcggacgtcctgccatggatgcagtgaaaaagggattgccgcacgcgccggaattgatcagatcc

SEQ ID NO: 71 - protein, 68 aa, synthetic construct
  REGION 1..68: note = Synthetic Construct
TPEQVVAIASNNGGRPALESIVAQLSRPDPALAALTNDHLVALACLGGRPAMDAVKKGLPHAPELIRS

SEQ ID NO: 72 - DNA, 1374 bp, synthetic construct
  misc_feature 1..1374: note = ND1-60-ND1
  source 1..1374: mol_type = other DNA
  CDS 1..1374
cttgttaagggcgaaatggagaaaaagaagtcagatctccgacacaagctgaaacatgtgccacatgagtacattgaactgatagagattgctcaggattccaaacagaaccggctttttgagttcaaggtggtagagtttcttaaggaagtgtatgactacaacgggaaacacctaggcgggtccagaaaacctgacggagctctgtataccaatgggctgaaaaccgactatgggatcatactagacacaaaggcctacaaggatgggtatagcctccctattagccaggccgatgagatgcagcggtacgttgacgaaaacaataaccgcaatgccatcattaaccccaacgagtggtggaaagtctacccgaattccatcctggactttaaattcttattcgtttctggcttctttaaaggcgactataagaaacagttagccagagtgtccaacctgaccaagaggaaaggagctgtcctcagtgtcgaacaattgctccttgggggcgaaaagatcaaggacggatctctgactttagaggacgtaggcgataaattcaacaacgatgagattatcttttacacccgggtgggcggcggcggctcaggcggcggcggctctggaggaggaggaagcggaggaggaggaagcgggggcggcggctctggcggcggcggcagcggaggaggaggatctggaggaggaggatccggcggcggcggcagcgggggaggagggagcggaggaggagggtccggaggaggcggcagcatgaccgcggtcctcgtgaaaggggagatggaaaagaagaagagtgacctgaggcacaaattgaaacacgttcctcacgagtacatcgagctgattgagattgcacaagattcgaagcagaatcgcctctttgagtttaaagtcgtcgaatttctcaaagaagtgtacgattacaatggtaagcatcttggtggatctcgcaagccagatggagccttgtacaccaatggcctgaagactgactatggcattatcctggatacgaaagcgtataaggacggctatagtctgccaatcagccaagcagatgaaatgcagagatacgtggatgaaaacaacaataggaatgccataatcaatcccaatgaatggtggaaggtgtatcccaacagcattctggacttcaagttcctgtttgtatctggtttcttcaagggagactacaagaaacagcttgcacgtgtcagcaacctgacaaaacggaagggtgctgtgttgtcagtggagcagctcttgctaggaggcgagaaaataaaggatggttcactgacactggaagacgtgggagataagttcaacaatgacgagatcatcttc

SEQ ID NO: 73 - protein, 458 aa, synthetic construct
  REGION 1..458: note = Synthetic Construct
LVKGEMEKKKSDLRHKLKHVPHEYIELIEIAQDSKQNRLFEFKVVEFLKEVYDYNGKHLGGSRKPDGALYTNGLKTDYGIILDTKAYKDGYSLPISQADEMQRYVDENNNRNAIINPNEWWKVYPNSILDFKFLFVSGFFKGDYKKQLARVSNLTKRKGAVLSVEQLLLGGEKIKDGSLTLEDVGDKFNNDEIIFYTRVGGGGSGGGGSGGGGSGGGGSGGGGSGGGGSGGGGSGGGGSGGGGSGGGGSGGGGSGGGGSMTAVLVKGEMEKKKSDLRHKLKHVPHEYIELIEIAQDSKQNRLFEFKVVEFLKEVYDYNGKHLGGSRKPDGALYTNGLKTDYGIILDTKAYKDGYSLPISQADEMQRYVDENNNRNAIINPNEWWKVYPNSILDFKFLFVSGFFKGDYKKQLARVSNLTKRKGAVLSVEQLLLGGEKIKDGSLTLEDVGDKFNNDEIIF

SEQ ID NO: 74 - DNA, 1566 bp, synthetic construct
  misc_feature 1..1566: note = ND1-120-ND1
  source 1..1566: mol_type = other DNA
  CDS 1..1566
cttgttaagggcgaaatggagaaaaagaagtcagatctccgacacaagctgaaacatgtgccacatgagtacattgaactgatagagattgctcaggattccaaacagaaccggctttttgagttcaaggtggtagagtttcttaaggaagtgtatgactacaacgggaaacacctaggcgggtccagaaaacctgacggagctctgtataccaatgggctgaaaaccgactatgggatcatactagacacaaaggcctacaaggatgggtatagcctccctattagccaggccgatgagatgcagcggtacgttgacgaaaacaataaccgcaatgccatcattaaccccaacgagtggtggaaagtctacccgaattccatcctggactttaaattcttattcgtttctggcttctttaaaggcgactataagaaacagttagccagagtgtccaacctgaccaagaggaaaggagctgtcctcagtgtcgaacaattgctccttgggggcgaaaagatcaaggacggatctctgactttagaggacgtaggcgataaattcaacaacgatgagattatcttttacacccgggtgggcggcggcggctcaggcggcggcggctctggaggaggaggaagcggaggaggaggaagcgggggcggcggctctggcggcggcggcagcggaggaggaggatctggaggaggaggatccggcggcggcggcagcgggggaggagggagcggaggaggagggtccggaggaggcggcagcatgaccggggtgggcggcggcggctcaggcggcggcggctctggaggaggaggaagcggaggaggaggaagcgggggcggcggctctggcggcggcggcagcggaggaggaggatctggaggaggaggatccggcggcggcggcagcgggggaggagggagcggaggaggagggtccggaggaggcggcagcatgaccgcggtcctcgtgaaaggggagatggaaaagaagaagagtgacctgaggcacaaattgaaacacgttcctcacgagtacatcgagctgattgagattgcacaagattcgaagcagaatcgcctctttgagtttaaagtcgtcgaatttctcaaagaagtgtacgattacaatggtaagcatcttggtggatctcgcaagccagatggagccttgtacaccaatggcctgaagactgactatggcattatcctggatacgaaagcgtataaggacggctatagtctgccaatcagccaagcagatgaaatgcagagatacgtggatgaaaacaacaataggaatgccataatcaatcccaatgaatggtggaaggtgtatcccaacagcattctggacttcaagttcctgtttgtatctggtttcttcaagggagactacaagaaacagcttgcacgtgtcagcaacctgacaaaacggaagggtgctgtgttgtcagtggagcagctcttgctaggaggcgagaaaataaaggatggttcactgacactggaagacgtgggagataagttcaacaatgacgagatcatcttc

SEQ ID NO: 75 - protein, 522 aa, synthetic construct
  REGION 1..522: note = Synthetic Construct
LVKGEMEKKKSDLRHKLKHVPHEYIELIEIAQDSKQNRLFEFKVVEFLKEVYDYNGKHLGGSRKPDGALYTNGLKTDYGIILDTKAYKDGYSLPISQADEMQRYVDENNNRNAIINPNEWWKVYPNSILDFKFLFVSGFFKGDYKKQLARVSNLTKRKGAVLSVEQLLLGGEKIKDGSLTLEDVGDKFNNDEIIFYTRVGGGGSGGGGSGGGGSGGGGSGGGGSGGGGSGGGGSGGGGSGGGGSGGGGSGGGGSGGGGSMTGVGGGGSGGGGSGGGGSGGGGSGGGGSGGGGSGGGGSGGGGSGGGGSGGGGSGGGGSGGGGSMTAVLVKGEMEKKKSDLRHKLKHVPHEYIELIEIAQDSKQNRLFEFKVVEFLKEVYDYNGKHLGGSRKPDGALYTNGLKTDYGIILDTKAYKDGYSLPISQADEMQRYVDENNNRNAIINPNEWWKVYPNSILDFKFLFVSGFFKGDYKKQLARVSNLTKRKGAVLSVEQLLLGGEKIKDGSLTLEDVGDKFNNDEIIF

SEQ ID NO: 76 - DNA, 1758 bp, synthetic construct
  misc_feature 1..1758: note = ND1-180-ND1
  source 1..1758: mol_type = other DNA
  CDS 1..1758
cttgttaagggcgaaatggagaaaaagaagtcagatctccgacacaagctgaaacatgtgccacatgagtacattgaactgatagagattgctcaggattccaaacagaaccggctttttgagttcaaggtggtagagtttcttaaggaagtgtatgactacaacgggaaacacctaggcgggtccagaaaacctgacggagctctgtataccaatgggctgaaaaccgactatgggatcatactagacacaaaggcctacaaggatgggtatagcctccctattagccaggccgatgagatgcagcggtacgttgacgaaaacaataaccgcaatgccatcattaaccccaacgagtggtggaaagtctacccgaattccatcctggactttaaattcttattcgtttctggcttctttaaaggcgactataagaaacagttagccagagtgtccaacctgaccaagaggaaaggagctgtcctcagtgtcgaacaattgctccttgggggcgaaaagatcaaggacggatctctgactttagaggacgtaggcgataaattcaacaacgatgagattatcttttacacccgggtgggcggcggcggctcaggcggcggcggctctggaggaggaggaagcggaggaggaggaagcgggggcggcggctctggcggcggcggcagcggaggaggaggatctggaggaggaggatccggcggcggcggcagcgggggaggagggagcggaggaggagggtccggaggaggcggcagcatgaccggggtgggcggcggcggctcaggcggcggcggctctggaggaggaggaagcggaggaggaggaagcgggggcggcggctctggcggcggcggcagcggaggaggaggatctggaggaggaggatccggcggcggcggcagcgggggaggagggagcggaggaggagggtccggaggaggcggcagcatgaccggggtgggcggcggcggctcaggcggcggcggctctggaggaggaggaagcggaggaggaggaagcgggggcggcggctctggcggcggcggcagcggaggaggaggatctggaggaggaggatccggcggcggcggcagcgggggaggagggagcggaggaggagggtccggaggaggcggcagcatgaccgcggtcctcgtgaaaggggagatggaaaagaagaagagtgacctgaggcacaaattgaaacacgttcctcacgagtacatcgagctgattgagattgcacaagattcgaagcagaatcgcctctttgagtttaaagtcgtcgaatttctcaaagaagtgtacgattacaatggtaagcatcttggtggatctcgcaagccagatggagccttgtacaccaatggcctgaagactgactatggcattatcctggatacgaaagcgtataaggacggctatagtctgccaatcagccaagcagatgaaatgcagagatacgtggatgaaaacaacaataggaatgccataatcaatcccaatgaatggtggaaggtgtatcccaacagcattctggacttcaagttcctgtttgtatctggtttcttcaagggagactacaagaaacagcttgcacgtgtcagcaacctgacaaaacggaagggtgctgtgttgtcagtggagcagctcttgctaggaggcgagaaaataaaggatggttcactgacactggaagacgtgggagataagttcaacaatgacgagatcatcttc

SEQ ID NO: 77 - protein, 586 aa, synthetic construct
  REGION 1..586: note = Synthetic Construct
LVKGEMEKKKSDLRHKLKHVPHEYIELIEIAQDSKQNRLFEFKVVEFLKEVYDYNGKHLGGSRKPDGALYTNGLKTDYGIILDTKAYKDGYSLPISQADEMQRYVDENNNRNAIINPNEWWKVYPNSILDFKFLFVSGFFKGDYKKQLARVSNLTKRKGAVLSVEQLLLGGEKIKDGSLTLEDVGDKFNNDEIIFYTRVGGGGSGGGGSGGGGSGGGGSGGGGSGGGGSGGGGSGGGGSGGGGSGGGGSGGGGSGGGGSMTGVGGGGSGGGGSGGGGSGGGGSGGGGSGGGGSGGGGSGGGGSGGGGSGGGGSGGGGSGGGGSMTGVGGGGSGGGGSGGGGSGGGGSGGGGSGGGGSGGGGSGGGGSGGGGSGGGGSGGGGSGGGGSMTAVLVKGEMEKKKSDLRHKLKHVPHEYIELIEIAQDSKQNRLFEFKVVEFLKEVYDYNGKHLGGSRKPDGALYTNGLKTDYGIILDTKAYKDGYSLPISQADEMQRYVDENNNRNAIINPNEWWKVYPNSILDFKFLFVSGFFKGDYKKQLARVSNLTKRKGAVLSVEQLLLGGEKIKDGSLTLEDVGDKFNNDEIIF

SEQ ID NO: 78 - DNA, 1479 bp, synthetic construct
  misc_feature 1..1479: note = ND1-95-ND1
  source 1..1479: mol_type = other DNA
  CDS 1..1479
cttgttaagggcgaaatggagaaaaagaagtcagatctccgacacaagctgaaacatgtgccacatgagtacattgaactgatagagattgctcaggattccaaacagaaccggctttttgagttcaaggtggtagagtttcttaaggaagtgtatgactacaacgggaaacacctaggcgggtccagaaaacctgacggagctctgtataccaatgggctgaaaaccgactatgggatcatactagacacaaaggcctacaaggatgggtatagcctccctattagccaggccgatgagatgcagcggtacgttgacgaaaacaataaccgcaatgccatcattaaccccaacgagtggtggaaagtctacccgaattccatcctggactttaaattcttattcgtttctggcttctttaaaggcgactataagaaacagttagccagagtgtccaacctgaccaagaggaaaggagctgtcctcagtgtcgaacaattgctccttgggggcgaaaagatcaaggacggatctctgactttagaggacgtaggcgataaattcaacaacgatgagattatcttttacacccgggtgggaagcggatccggatctggaagcatcaccaggaccacaaaccctcgcaatgtggtgccaaagatctacatgtccgccggctctatccctctgaccacacacatcacaaacagcatccagccaaccctgtggacaatcggatccatcaatggagtggcaccactggccaagtctatcaagctgggcatccctgtgaccggcagcgcctacacagaccagaccacagccatggtgcggaagaaggtgagcgtgttcatgggcagcggatctggaagcggatctagcatgaccgcggtcctcgtgaaaggggagatggaaaagaagaagagtgacctgaggcacaaattgaaacacgttcctcacgagtacatcgagctgattgagattgcacaagattcgaagcagaatcgcctctttgagtttaaagtcgtcgaatttctcaaagaagtgtacgattacaatggtaagcatcttggtggatctcgcaagccagatggagccttgtacaccaatggcctgaagactgactatggcattatcctggatacgaaagcgtataaggacggctatagtctgccaatcagccaagcagatgaaatgcagagatacgtggatgaaaacaacaataggaatgccataatcaatcccaatgaatggtggaaggtgtatcccaacagcattctggacttcaagttcctgtttgtatctggtttcttcaagggagactacaagaaacagcttgcacgtgtcagcaacctgacaaaacggaagggtgctgtgttgtcagtggagcagctcttgctaggaggcgagaaaataaaggatggttcactgacactggaagacgtgggagataagttcaacaatgacgagatcatcttc

SEQ ID NO: 79 - protein, 493 aa, synthetic construct
  REGION 1..493: note = Synthetic Construct
LVKGEMEKKKSDLRHKLKHVPHEYIELIEIAQDSKQNRLFEFKVVEFLKEVYDYNGKHLGGSRKPDGALYTNGLKTDYGIILDTKAYKDGYSLPISQADEMQRYVDENNNRNAIINPNEWWKVYPNSILDFKFLFVSGFFKGDYKKQLARVSNLTKRKGAVLSVEQLLLGGEKIKDGSLTLEDVGDKFNNDEIIFYTRVGSGSGSGSITRTTNPRNVVPKIYMSAGSIPLTTHITNSIQPTLWTIGSINGVAPLAKSIKLGIPVTGSAYTDQTTAMVRKKVSVFMGSGSGSGSSMTAVLVKGEMEKKKSDLRHKLKHVPHEYIELIEIAQDSKQNRLFEFKVVEFLKEVYDYNGKHLGGSRKPDGALYTNGLKTDYGIILDTKAYKDGYSLPISQADEMQRYVDENNNRNAIINPNEWWKVYPNSILDFKFLFVSGFFKGDYKKQLARVSNLTKRKGAVLSVEQLLLGGEKIKDGSLTLEDVGDKFNNDEIIF

SEQ ID NO: 80 - DNA, 1350 bp, synthetic construct
  misc_feature 1..1350: note = ND2-60-ND2
  source 1..1350: mol_type = other DNA
  CDS 1..1350
attgttaagagcagcattgagatgagcaaggccaatatgagggataacctacagatgctcccacacgactacatcgagcttatcgagatctctcaggatccttatcaaaaccgcatcttcgaaatgaaagtgatggatctgtttatcaacgaatatggcttcagtgggtcacatctgggaggctccagaaaaccagatggagccatgtatgcccatgggtttggggtgatcgtggacactaaggcgtataaggatggatacaatctccccatatcccaggctgacgaaatggagcgctatgtcagggaaaacatcgaccggaatgagcacgtgaattccaataggtggtggaatatttttccggaagataccaatgagtacaagttcttgtttgtgtctgggttcttcaagggcaatttcgagaagcagctagaacggatttccatcgacacaggggttcaaggaggagctctgtcagtggagcacctgctgctgggggctgaatacataaaacgaggcattcttacactgtatgacttcaagaattcgtttctgaacaaagagatccagttctacacccgggtgggcggcggcggctcaggcggcggcggctctggaggaggaggaagcggaggaggaggaagcgggggcggcggctctggcggcggcggcagcggaggaggaggatctggaggaggaggatccggcggcggcggcagcgggggaggagggagcggaggaggagggtccggaggaggcggcagcatgaccgcggtcattgtgaagtctagtatcgaaatgtccaaagccaatatgcgcgacaatctccagatgcttccccatgactatatcgaactgatcgaaatctcccaagacccttaccagaaccggatatttgagatgaaggtaatggacctgttcattaacgagtatggctttagcggcagtcatctcggtggaagcaggaagcctgatggtgccatgtacgctcacggatttggcgtcattgtcgataccaaagcatacaaggatgggtacaacttgcccataagtcaggccgatgagatggaaagatacgtgagagagaacattgaccgtaacgagcacgtcaatagcaaccgatggtggaacatctttccagaggataccaacgaatacaaattcctctttgtgtcaggtttctttaagggcaactttgaaaaacagcttgagcggatctcaattgacactggcgtacaaggtggcgcattatctgttgaacacttgttactgggagcagagtatattaaaagaggtatattgacgctctacgacttcaaaaactctttcctgaataaggagattcagttc

SEQ ID NO: 81 - protein, 450 aa, synthetic construct
  REGION 1..450: note = Synthetic Construct
IVKSSIEMSKANMRDNLQMLPHDYIELIEISQDPYQNRIFEMKVMDLFINEYGFSGSHLGGSRKPDGAMYAHGFGVIVDTKAYKDGYNLPISQADEMERYVRENIDRNEHVNSNRWWNIFPEDTNEYKFLFVSGFFKGNFEKQLERISIDTGVQGGALSVEHLLLGAEYIKRGILTLYDFKNSFLNKEIQFYTRVGGGGSGGGGSGGGGSGGGGSGGGGSGGGGSGGGGSGGGGSGGGGSGGGGSGGGGSGGGGSMTAVIVKSSIEMSKANMRDNLQMLPHDYIELIEISQDPYQNRIFEMKVMDLFINEYGFSGSHLGGSRKPDGAMYAHGFGVIVDTKAYKDGYNLPISQADEMERYVRENIDRNEHVNSNRWWNIFPEDTNEYKFLFVSGFFKGNFEKQLERISIDTGVQGGALSVEHLLLGAEYIKRGILTLYDFKNSFLNKEIQF

SEQ ID NO: 82 - DNA, 1542 bp, synthetic construct
  misc_feature 1..1542: note = ND2-120-ND2
  source 1..1542: mol_type = other DNA
  CDS 1..1542
attgttaagagcagcattgagatgagcaaggccaatatgagggataacctacagatgctcccacacgactacatcgagcttatcgagatctctcaggatccttatcaaaaccgcatcttcgaaatgaaagtgatggatctgtttatcaacgaatatggcttcagtgggtcacatctgggaggctccagaaaaccagatggagccatgtatgcccatgggtttggggtgatcgtggacactaaggcgtataaggatggatacaatctccccatatcccaggctgacgaaatggagcgctatgtcagggaaaacatcgaccggaatgagcacgtgaattccaataggtggtggaatatttttccggaagataccaatgagtacaagttcttgtttgtgtctgggttcttcaagggcaatttcgagaagcagctagaacggatttccatcgacacaggggttcaaggaggagctctgtcagtggagcacctgctgctgggggctgaatacataaaacgaggcattcttacactgtatgacttcaagaattcgtttctgaacaaagagatccagttctacacccgggtgggcggcggcggctcaggcggcggcggctctggaggaggaggaagcggaggaggaggaagcgggggcggcggctctggcggcggcggcagcggaggaggaggatctggaggaggaggatccggcggcggcggcagcgggggaggagggagcggaggaggagggtccggaggaggcggcagcatgaccggggtgggcggcggcggctcaggcggcggcggctctggaggaggaggaagcggaggaggaggaagcgggggcggcggctctggcggcggcggcagcggaggaggaggatctggaggaggaggatccggcggcggcggcagcgggggaggagggagcggaggaggagggtccggaggaggcggcagcatgaccgcggtcattgtgaagtctagtatcgaaatgtccaaagccaatatgcgcgacaatctccagatgcttccccatgactatatcgaactgatcgaaatctcccaagacccttaccagaaccggatatttgagatgaaggtaatggacctgttcattaacgagtatggctttagcggcagtcatctcggtggaagcaggaagcctgatggtgccatgtacgctcacggatttggcgtcattgtcgataccaaagcatacaaggatgggtacaacttgcccataagtcaggccgatgagatggaaagatacgtgagagagaacattgaccgtaacgagcacgtcaatagcaaccgatggtggaacatctttccagaggataccaacgaatacaaattcctctttgtgtcaggtttctttaagggcaactttgaaaaacagcttgagcggatctcaattgacactggcgtacaaggtggcgcattatctgttgaacacttgttactgggagcagagtatattaaaagaggtatattgacgctctacgacttcaaaaactctttcctgaataaggagattcagttc

SEQ ID NO: 83 - protein, 514 aa, synthetic construct
  REGION 1..514: note = Synthetic Construct
IVKSSIEMSKANMRDNLQMLPHDYIELIEISQDPYQNRIFEMKVMDLFINEYGFSGSHLGGSRKPDGAMYAHGFGVIVDTKAYKDGYNLPISQADEMERYVRENIDRNEHVNSNRWWNIFPEDTNEYKFLFVSGFFKGNFEKQLERISIDTGVQGGALSVEHLLLGAEYIKRGILTLYDFKNSFLNKEIQFYTRVGGGGSGGGGSGGGGSGGGGSGGGGSGGGGSGGGGSGGGGSGGGGSGGGGSGGGGSGGGGSMTGVGGGGSGGGGSGGGGSGGGGSGGGGSGGGGSGGGGSGGGGSGGGGSGGGGSGGGGSGGGGSMTAVIVKSSIEMSKANMRDNLQMLPHDYIELIEISQDPYQNRIFEMKVMDLFINEYGFSGSHLGGSRKPDGAMYAHGFGVIVDTKAYKDGYNLPISQADEMERYVRENIDRNEHVNSNRWWNIFPEDTNEYKFLFVSGFFKGNFEKQLERISIDTGVQGGALSVEHLLLGAEYIKRGILTLYDFKNSFLNKEIQF

SEQ ID NO: 84 - DNA, 1734 bp, synthetic construct
  misc_feature 1..1734: note = ND2-180-ND2
  source 1..1734: mol_type = other DNA
  CDS 1..1734
attgttaagagcagcattgagatgagcaaggccaatatgagggataacctacagatgctcccacacgactacatcgagcttatcgagatctctcaggatccttatcaaaaccgcatcttcgaaatgaaagtgatggatctgtttatcaacgaatatggcttcagtgggtcacatctgggaggctccagaaaaccagatggagccatgtatgcccatgggtttggggtgatcgtggacactaaggcgtataaggatggatacaatctccccatatcccaggctgacgaaatggagcgctatgtcagggaaaacatcgaccggaatgagcacgtgaattccaataggtggtggaatatttttccggaagataccaatgagtacaagttcttgtttgtgtctgggttcttcaagggcaatttcgagaagcagctagaacggatttccatcgacacaggggttcaaggaggagctctgtcagtggagcacctgctgctgggggctgaatacataaaacgaggcattcttacactgtatgacttcaagaattcgtttctgaacaaagagatccagttctacacccgggtgggcggcggcggctcaggcggcggcggctctggaggaggaggaagcggaggaggaggaagcgggggcggcggctctggcggcggcggcagcggaggaggaggatctggaggaggaggatccggcggcggcggcagcgggggaggagggagcggaggaggagggtccggaggaggcggcagcatgaccggggtgggcggcggcggctcaggcggcggcggctctggaggaggaggaagcggaggaggaggaagcgggggcggcggctctggcggcggcggcagcggaggaggaggatctggaggaggaggatccggcggcggcggcagcgggggaggagggagcggaggaggagggtccggaggaggcggcagcatgaccggggtgggcggcggcggctcaggcggcggcggctctggaggaggaggaagcggaggaggaggaagcgggggcggcggctctggcggcggcggcagcggaggaggaggatctggaggaggaggatccggcggcggcggcagcgggggaggagggagcggaggaggagggtccggaggaggcggcagcatgaccgcggtcattgtgaagtctagtatcgaaatgtccaaagccaatatgcgcgacaatctccagatgcttccccatgactatatcgaactgatcgaaatctcccaagacccttaccagaaccggatatttgagatgaaggtaatggacctgttcattaacgagtatggctttagcggcagtcatctcggtggaagcaggaagcctgatggtgccatgtacgctcacggatttggcgtcattgtcgataccaaagcatacaaggatgggtacaacttgcccataagtcaggccgatgagatggaaagatacgtgagagagaacattgaccgtaacgagcacgtcaatagcaaccgatggtggaacatctttccagaggataccaacgaatacaaattcctctttgtgtcaggtttctttaagggcaactttgaaaaacagcttgagcggatctcaattgacactggcgtacaaggtggcgcattatctgttgaacacttgttactgggagcagagtatattaaaagaggtatattgacgctctacgacttcaaaaactctttcctgaataaggagattcagttc

SEQ ID NO: 85 - protein, 578 aa, synthetic construct
  REGION 1..578: note = Synthetic Construct
IVKSSIEMSKANMRDNLQMLPHDYIELIEISQDPYQNRIFEMKVMDLFINEYGFSGSHLGGSRKPDGAMYAHGFGVIVDTKAYKDGYNLPISQADEMERYVRENIDRNEHVNSNRWWNIFPEDTNEYKFLFVSGFFKGNFEKQLERISIDTGVQGGALSVEHLLLGAEYIKRGILTLYDFKNSFLNKEIQFYTRVGGGGSGGGGSGGGGSGGGGSGGGGSGGGGSGGGGSGGGGSGGGGSGGGGSGGGGSGGGGSMTGVGGGGSGGGGSGGGGSGGGGSGGGGSGGGGSGGGGSGGGGSGGGGSGGGGSGGGGSGGGGSMTGVGGGGSGGGGSGGGGSGGGGSGGGGSGGGGSGGGGSGGGGSGGGGSGGGGSGGGGSGGGGSMTAVIVKSSIEMSKANMRDNLQMLPHDYIELIEISQDPYQNRIFEMKVMDLFINEYGFSGSHLGGSRKPDGAMYAHGFGVIVDTKAYKDGYNLPISQADEMERYVRENIDRNEHVNSNRWWNIFPEDTNEYKFLFVSGFFKGNFEKQLERISIDTGVQGGALSVEHLLLGAEYIKRGILTLYDFKNSFLNKEIQF

SEQ ID NO: 86 - DNA, 1455 bp, synthetic construct
  misc_feature 1..1455: note = ND2-95-ND2
  source 1..1455: mol_type = other DNA
  CDS 1..1455
attgttaagagcagcattgagatgagcaaggccaatatgagggataacctacagatgctcccacacgactacatcgagcttatcgagatctctcaggatccttatcaaaaccgcatcttcgaaatgaaagtgatggatctgtttatcaacgaatatggcttcagtgggtcacatctgggaggctccagaaaaccagatggagccatgtatgcccatgggtttggggtgatcgtggacactaaggcgtataaggatggatacaatctccccatatcccaggctgacgaaatggagcgctatgtcagggaaaacatcgaccggaatgagcacgtgaattccaataggtggtggaatatttttccggaagataccaatgagtacaagttcttgtttgtgtctgggttcttcaagggcaatttcgagaagcagctagaacggatttccatcgacacaggggttcaaggaggagctctgtcagtggagcacctgctgctgggggctgaatacataaaacgaggcattcttacactgtatgacttcaagaattcgtttctgaacaaagagatccagttctacacccgggtgggaagcggatccggatctggaagcatcaccaggaccacaaaccctcgcaatgtggtgccaaagatctacatgtccgccggctctatccctctgaccacacacatcacaaacagcatccagccaaccctgtggacaatcggatccatcaatggagtggcaccactggccaagtctatcaagctgggcatccctgtgaccggcagcgcctacacagaccagaccacagccatggtgcggaagaaggtgagcgtgttcatgggcagcggatctggaagcggatctagcatgaccgcggtcattgtgaagtctagtatcgaaatgtccaaagccaatatgcgcgacaatctccagatgcttccccatgactatatcgaactgatcgaaatctcccaagacccttaccagaaccggatatttgagatgaaggtaatggacctgttcattaacgagtatggctttagcggcagtcatctcggtggaagcaggaagcctgatggtgccatgtacgctcacggatttggcgtcattgtcgataccaaagcatacaaggatgggtacaacttgcccataagtcaggccgatgagatggaaagatacgtgagagagaacattgaccgtaacgagcacgtcaatagcaaccgatggtggaacatctttccagaggataccaacgaatacaaattcctctttgtgtcaggtttctttaagggcaactttgaaaaacagcttgagcggatctcaattgacactggcgtacaaggtggcgcattatctgttgaacacttgttactgggagcagagtatattaaaagaggtatattgacgctctacgacttcaaaaactctttcctgaataaggagattcagttc

SEQ ID NO: 87 - protein, 485 aa, synthetic construct
  REGION 1..485: note = Synthetic Construct
IVKSSIEMSKANMRDNLQMLPHDYIELIEISQDPYQNRIFEMKVMDLFINEYGFSGSHLGGSRKPDGAMYAHGFGVIVDTKAYKDGYNLPISQADEMERYVRENIDRNEHVNSNRWWNIFPEDTNEYKFLFVSGFFKGNFEKQLERISIDTGVQGGALSVEHLLLGAEYIKRGILTLYDFKNSFLNKEIQFYTRVGSGSGSGSITRTTNPRNVVPKIYMSAGSIPLTTHITNSIQPTLWTIGSINGVAPLAKSIKLGIPVTGSAYTDQTTAMVRKKVSVFMGSGSGSGSSMTAVIVKSSIEMSKANMRDNLQMLPHDYIELIEISQDPYQNRIFEMKVMDLFINEYGFSGSHLGGSRKPDGAMYAHGFGVIVDTKAYKDGYNLPISQADEMERYVRENIDRNEHVNSNRWWNIFPEDTNEYKFLFVSGFFKGNFEKQLERISIDTGVQGGALSVEHLLLGAEYIKRGILTLYDFKNSFLNKEIQF

SEQ ID NO: 88 - DNA, 1497 bp, synthetic construct
  misc_feature 1..1497: note = ND1-GSSx32-ND1
  source 1..1497: mol_type = other DNA
  CDS 1..1497
cttgttaagggcgaaatggagaaaaagaagtcagatctccgacacaagctgaaacatgtgccacatgagtacattgaactgatagagattgctcaggattccaaacagaaccggctttttgagttcaaggtggtagagtttcttaaggaagtgtatgactacaacgggaaacacctaggcgggtccagaaaacctgacggagctctgtataccaatgggctgaaaaccgactatgggatcatactagacacaaaggcctacaaggatgggtatagcctccctattagccaggccgatgagatgcagcggtacgttgacgaaaacaataaccgcaatgccatcattaaccccaacgagtggtggaaagtctacccgaattccatcctggactttaaattcttattcgtttctggcttctttaaaggcgactataagaaacagttagccagagtgtccaacctgaccaagaggaaaggagctgtcctcagtgtcgaacaattgctccttgggggcgaaaagatcaaggacggatctctgactttagaggacgtaggcgataaattcaacaacgatgagattatcttttacacccgggtggggtctagtggctccagcggatcaagtggcagctccgggtctagtggctccagcggatcaagtgggagttctggcagctcaggatctagtggcagctccgggtctagtggctccagcggatcaagtgggagttctggcagctcaggatctagtggcagctccgggtctagtggctccagcggatcaagtgggagttctggcagctcaggatctagtggcagctccgggtctagtggctccagcggatcaagtgggagttctggcagctcaggatctagtggcagctccggaggaggcggcagcatgaccgcggtcctcgtgaaaggggagatggaaaagaagaagagtgacctgaggcacaaattgaaacacgttcctcacgagtacatcgagctgattgagattgcacaagattcgaagcagaatcgcctctttgagtttaaagtcgtcgaatttctcaaagaagtgtacgattacaatggtaagcatcttggtggatctcgcaagccagatggagccttgtacaccaatggcctgaagactgactatggcattatcctggatacgaaagcgtataaggacggctatagtctgccaatcagccaagcagatgaaatgcagagatacgtggatgaaaacaacaataggaatgccataatcaatcccaatgaatggtggaaggtgtatcccaacagcattctggacttcaagttcctgtttgtatctggtttcttcaagggagactacaagaaacagcttgcacgtgtcagcaacctgacaaaacggaagggtgctgtgttgtcagtggagcagctcttgctaggaggcgagaaaataaaggatggttcactgacactggaagacgtgggagataagttcaacaatgacgagatcatcttc

SEQ ID NO: 89 - protein, 499 aa, synthetic construct
  REGION 1..499: note = Synthetic Construct
LVKGEMEKKKSDLRHKLKHVPHEYIELIEIAQDSKQNRLFEFKVVEFLKEVYDYNGKHLGGSRKPDGALYTNGLKTDYGIILDTKAYKDGYSLPISQADEMQRYVDENNNRNAIINPNEWWKVYPNSILDFKFLFVSGFFKGDYKKQLARVSNLTKRKGAVLSVEQLLLGGEKIKDGSLTLEDVGDKFNNDEIIFYTRVGSSGSSGSSGSSGSSGSSGSSGSSGSSGSSGSSGSSGSSGSSGSSGSSGSSGSSGSSGSSGSSGSSGSSGSSGSSGSSGSSGSSGSSGSSGSSGSSGGGGSMTAVLVKGEMEKKKSDLRHKLKHVPHEYIELIEIAQDSKQNRLFEFKVVEFLKEVYDYNGKHLGGSRKPDGALYTNGLKTDYGIILDTKAYKDGYSLPISQADEMQRYVDENNNRNAIINPNEWWKVYPNSILDFKFLFVSGFFKGDYKKQLARVSNLTKRKGAVLSVEQLLLGGEKIKDGSLTLEDVGDKFNNDEIIF

SEQ ID NO: 90 - DNA, 1485 bp, synthetic construct
  misc_feature 1..1485: note = ND1-SAGGx24-ND1
  source 1..1485: mol_type = other DNA
  CDS 1..1485
cttgttaagggcgaaatggagaaaaagaagtcagatctccgacacaagctgaaacatgtgccacatgagtacattgaactgatagagattgctcaggattccaaacagaaccggctttttgagttcaaggtggtagagtttcttaaggaagtgtatgactacaacgggaaacacctaggcgggtccagaaaacctgacggagctctgtataccaatgggctgaaaaccgactatgggatcatactagacacaaaggcctacaaggatgggtatagcctccctattagccaggccgatgagatgcagcggtacgttgacgaaaacaataaccgcaatgccatcattaaccccaacgagtggtggaaagtctacccgaattccatcctggactttaaattcttattcgtttctggcttctttaaaggcgactataagaaacagttagccagagtgtccaacctgaccaagaggaaaggagctgtcctcagtgtcgaacaattgctccttgggggcgaaaagatcaaggacggatctctgactttagaggacgtaggcgataaattcaacaacgatgagattatcttttacacccgggtgtctgctggcgggtccgccgggggcagtgctggcggatctgctggcgggtccgccgggggcagtgctggcggatctgctggcgggtccgccgggggcagtgctggcggatctgctggcgggtccgccgggggcagtgctggcggatctgctggcgggtccgccgggggcagtgctggcggatctgctggcgggtccgccgggggcagtgctggcggatctgctggcgggtccgccgggggcagtgctggcggatctgctggcgggtccgccgggggcagtgctggcggatccatgaccgcggtcctcgtgaaaggggagatggaaaagaagaagagtgacctgaggcacaaattgaaacacgttcctcacgagtacatcgagctgattgagattgcacaagattcgaagcagaatcgcctctttgagtttaaagtcgtcgaatttctcaaagaagtgtacgattacaatggtaagcatcttggtggatctcgcaagccagatggagccttgtacaccaatggcctgaagactgactatggcattatcctggatacgaaagcgtataaggacggctatagtctgccaatcagccaagcagatgaaatgcagagatacgtggatgaaaacaacaataggaatgccataatcaatcccaatgaatggtggaaggtgtatcccaacagcattctggacttcaagttcctgtttgtatctggtttcttcaagggagactacaagaaacagcttgcacgtgtcagcaacctgacaaaacggaagggtgctgtgttgtcagtggagcagctcttgctaggaggcgagaaaataaaggatggttcactgacactggaagacgtgggagataagttcaacaatgacgagatcatcttc

SEQ ID NO: 91 - protein, 495 aa, synthetic construct
  REGION 1..495: note = Synthetic Construct
LVKGEMEKKKSDLRHKLKHVPHEYIELIEIAQDSKQNRLFEFKVVEFLKEVYDYNGKHLGGSRKPDGALYTNGLKTDYGIILDTKAYKDGYSLPISQADEMQRYVDENNNRNAIINPNEWWKVYPNSILDFKFLFVSGFFKGDYKKQLARVSNLTKRKGAVLSVEQLLLGGEKIKDGSLTLEDVGDKFNNDEIIFYTRVSAGGSAGGSAGGSAGGSAGGSAGGSAGGSAGGSAGGSAGGSAGGSAGGSAGGSAGGSAGGSAGGSAGGSAGGSAGGSAGGSAGGSAGGSAGGSAGGSMTAVLVKGEMEKKKSDLRHKLKHVPHEYIELIEIAQDSKQNRLFEFKVVEFLKEVYDYNGKHLGGSRKPDGALYTNGLKTDYGIILDTKAYKDGYSLPISQADEMQRYVDENNNRNAIINPNEWWKVYPNSILDFKFLFVSGFFKGDYKKQLARVSNLTKRKGAVLSVEQLLLGGEKIKDGSLTLEDVGDKFNNDEIIF

SEQ ID NO: 92 - DNA, 1482 bp, synthetic construct
  misc_feature 1..1482: note = ND1-GGGGSx19-ND1
  source 1..1482: mol_type = other DNA
  CDS 1..1482
cttgttaagggcgaaatggagaaaaagaagtcagatctccgacacaagctgaaacatgtgccacatgagtacattgaactgatagagattgctcaggattccaaacagaaccggctttttgagttcaaggtggtagagtttcttaaggaagtgtatgactacaacgggaaacacctaggcgggtccagaaaacctgacggagctctgtataccaatgggctgaaaaccgactatgggatcatactagacacaaaggcctacaaggatgggtatagcctccctattagccaggccgatgagatgcagcggtacgttgacgaaaacaataaccgcaatgccatcattaaccccaacgagtggtggaaagtctacccgaattccatcctggactttaaattcttattcgtttctggcttctttaaaggcgactataagaaacagttagccagagtgtccaacctgaccaagaggaaaggagctgtcctcagtgtcgaacaattgctccttgggggcgaaaagatcaaggacggatctctgactttagaggacgtaggcgataaattcaacaacgatgagattatcttttacacccgggtggggggcggagggtctggcggagggggctctggagggggcggatccgggggcggagggtctggcggagggggctctggagggggcggatccgggggcggagggtctggcggagggggctctggagggggcggatccgggggcggagggtctggcggagggggctctggagggggcggatccgggggcggagggtctggcggagggggctctggagggggcggatccgggggcggagggtctggcggagggggctctggagggggcggatcagggggcggagggtccggaatgaccgcggtcctcgtgaaaggggagatggaaaagaagaagagtgacctgaggcacaaattgaaacacgttcctcacgagtacatcgagctgattgagattgcacaagattcgaagcagaatcgcctctttgagtttaaagtcgtcgaatttctcaaagaagtgtacgattacaatggtaagcatcttggtggatctcgcaagccagatggagccttgtacaccaatggcctgaagactgactatggcattatcctggatacgaaagcgtataaggacggctatagtctgccaatcagccaagcagatgaaatgcagagatacgtggatgaaaacaacaataggaatgccataatcaatcccaatgaatggtggaaggtgtatcccaacagcattctggacttcaagttcctgtttgtatctggtttcttcaagggagactacaagaaacagcttgcacgtgtcagcaacctgacaaaacggaagggtgctgtgttgtcagtggagcagctcttgctaggaggcgagaaaataaaggatggttcactgacactggaagacgtgggagataagttcaacaatgacgagatcatcttc

SEQ ID NO: 93 - protein, 494 aa, synthetic construct
  REGION 1..494: note = Synthetic Construct
LVKGEMEKKKSDLRHKLKHVPHEYIELIEIAQDSKQNRLFEFKVVEFLKEVYDYNGKHLGGSRKPDGALYTNGLKTDYGIILDTKAYKDGYSLPISQADEMQRYVDENNNRNAIINPNEWWKVYPNSILDFKFLFVSGFFKGDYKKQLARVSNLTKRKGAVLSVEQLLLGGEKIKDGSLTLEDVGDKFNNDEIIFYTRVGGGGSGGGGSGGGGSGGGGSGGGGSGGGGSGGGGSGGGGSGGGGSGGGGSGGGGSGGGGSGGGGSGGGGSGGGGSGGGGSGGGGSGGGGSGGGGSGMTAVLVKGEMEKKKSDLRHKLKHVPHEYIELIEIAQDSKQNRLFEFKVVEFLKEVYDYNGKHLGGSRKPDGALYTNGLKTDYGIILDTKAYKDGYSLPISQADEMQRYVDENNNRNAIINPNEWWKVYPNSILDFKFLFVSGFFKGDYKKQLARVSNLTKRKGAVLSVEQLLLGGEKIKDGSLTLEDVGDKFNNDEIIF

SEQ ID NO: 94 - DNA, 237 bp, synthetic construct
  misc_feature 1..237: note = EGxAPCxFP
  source 1..237: mol_type = other DNA
ctcgatgctgttcccaggtactgttgttggctgttggtgaggaaggtgaagcactcagttgccttctcgggcctcggcgccccctatgtacgcctccctgggctcgggtccggtcgcccctttgcccgcttctgtaccaccctcagttctcgggtcctggagcaccggcggcagcaggagctgcgtccggcaggagacgaagagcccgggcggcgctcgtacttctggccactgggc

SEQ ID NO: 95 - DNA, 433 bp, synthetic construct
  misc_feature 1..433: note = EGxRosa26xFP
  source 1..433: mol_type = other DNA
gggagaaggccgcaccctactcggctgggggaggggagtgccgcaatacctttctgggagttctctgctgcctcctgtcttctaaagaccgccccgggactggaaggatcccttccccctttcccctcgtgatctgcaagtcgaggctttctgggagatgggcgggagtcttctgggcaggcttgagggctaacctggtgcgtgggcgttgtcctgcaggggaattgaactggtgtaaaattggaagggtgagaattcccacggattttcgtttgtgtcgggaggtgattgtaataggggcaaaggagggaaatgggagactaggtgctcgcctggggttttgtgcagcaaaactacaggttattattaataagccttggagtatttttcatcgagttggattaaggtcatgctcacccgagttttatgctca

SEQ ID NO: 96 - DNA, 721 bp, synthetic construct
  misc_feature 1..721: note = EGxHPRT1xFP
  source 1..721: mol_type = other DNA
gacacacatatgcacttgcatttgcccccacaatgctcaaacatactcaatgtgtagagtagaaactgcgtagactagtctctgatgtttaaagtatttttgccacatttgtcatacctctttaaattgttatctttttctacttgtgacctgaaggaagaggattatagtttattacaaaaatataaaattaactgcccttcataccctctcatacccaaattcctctggcgaactaaggcttattttctaaattttgttaaatatggatatcttatgctctgatttgaaacagctgtctttctttttcagattagtgatgatgaaccaggctatgacctagatttattttgtattcctaatcactatgtcgaggatttggaaaaggtgtttattcctcatggagtgattatggacaggtaagtaagatcttaattgaaggggctggagagatggctcagcggttaagagcactgactgctcttccagaggttctgagttcaattcccagcaaccacatgatggctcacaaccatccctaatgagatctggtgccctcttctggcctgcagggacacatgcagacagaacagatcttaattgaagttttatgggtttattttagatgtgtctgtgtatgtttgtgataggcatgtatttgatacatatgtataatgtatatatttatgtaaaagctagagaaggacattgggtgccatac

SEQ ID NO: 97 - protein, 585 aa, Bacillus sp. SGD-V-76
MATKRVVRTFGWIQNPGKFENLKRTVQVFDENSKVYKEVRDIKIPNLVKDKDVRTTLIAAMNRLENYYSYKELVGTGTSVRAQAPCDAIIQAAIQDQGNKKGYIDNWSSDGFVRWAHALGFLEYNSDKDSFYLTDIGLEYSRSTDDSLNEKIILIEALSSYPPAIRILTLLENGEHLTKFDLGKQLGFSGESGFTSLPQNLFLDALANAPSSPPTIKNSIRSDWEGSADKYARMISGWLVKMGLVAQGRKNFVVPTVGGSTRNEYISHAFKITKDGLDVLRRAKGASKHVRVPKRVYWEMFATNINDRVYVRTRRAYTLYLLMRSNTALNTVQLQVKLKALGFEELEETIENDVKGLINSGIFINVTNKGYHFKDTIKPFEIPEFGVTEPLVKGEMEKKKSDLRHKLKHVPHEYIELIEIAQDSKQNRLFEFKVVEFLKEVYDYNGKHLGGSRKPDGALYTNGLKTDYGIILDTKAYKDGYSLPISQADEMQRYVDENNNRNAIINPNEWWKVYPNSILDFKFLFVSGFFKGDYKKQLARVSNLTKRKGAVLSVEQLLLGGEKIKDGSLTLEDVGDKFNNDEIIF

SEQ ID NO: 98 - protein, 195 aa, synthetic construct
LVKGEMEKKKSDLRHKLKHVPHEYIELIEIAQDSKQNRLFEFKVVEFLKEVYDYNGKHLGGSRKPDGALYTNGLKTDYGIILDTKAYKDGYSLPISQADEMQRYVDENNNRNAIINPNEWWKVYPNSILDFKFLFVSGFFKGDYKKQLARVSNLTKRKGAVLSVEQLLLGGEKIKDGSLTLEDVGDKFNNDEIIF

SEQ ID NO: 99 - protein, 5 aa, synthetic construct
GGGGS

SEQ ID NO: 100 - DNA, 27 bp, synthetic construct
  source 1..27: mol_type = other DNA; note = TALEvector_F
gaattctgcagatatccagcacagtgg

SEQ ID NO: 101 - DNA, 32 bp, synthetic construct
  source 1..32: mol_type = other DNA; note = ND1-N_R_infEcoRI
atatctgcagaattccccacccgggtgtaaaa

SEQ ID NO: 102 - DNA, 39 bp, synthetic construct
  source 1..39: mol_type = other DNA; note = ND1-C_F_infT7
actcactatagggaggattatcttttacacccgggtggg

SEQ ID NO: 103 - DNA, 28 bp, synthetic construct
  source 1..28: mol_type = other DNA; note = T7-L_R
ctccctatagtgagtcgtattaatttcg

SEQ ID NO: 104 - DNA, 27 bp, synthetic construct
  source 1..27: mol_type = other DNA; note = ND1-N-D450N_F
aacggagctctgtataccaatgggctg

SEQ ID NO: 105 - DNA, 28 bp, synthetic construct
  source 1..28: mol_type = other DNA; note = ND1-N-D450N_R
atacagagctccgttaggttttctggac

SEQ ID NO: 106 - DNA, 27 bp, synthetic construct
  source 1..27: mol_type = other DNA; note = ND1-N-D450A_F
gccggagctctgtataccaatgggctg

SEQ ID NO: 107 - DNA, 28 bp, synthetic construct
  source 1..28: mol_type = other DNA; note = ND1-N-D450A_R
atacagagctccggcaggttttctggac

SEQ ID NO: 108 - DNA, 29 bp, synthetic construct
  source 1..29: mol_type = other DNA; note = ND1-N-D467A_F
gccacaaaggcctacaaggatgggtatag

SEQ ID NO: 109 - DNA, 27 bp, synthetic construct
  source 1..27: mol_type = other DNA; note = ND1-N-D467A_R
gtaggcctttgtggctagtatgatccc

SEQ ID NO: 110 - DNA, 27 bp, synthetic construct
  source 1..27: mol_type = other DNA; note = ND1-C-D450N_F
caaatggagccttgtacaccaatggcc

SEQ ID NO: 111 - DNA, 27 bp, synthetic construct
  source 1..27: mol_type = other DNA; note = ND1-C-D450N_R
acaaggctccatttggcttgcgagatc

SEQ ID NO: 112 - DNA, 27 bp, synthetic construct
  source 1..27: mol_type = other DNA; note = ND1-C-D450A_F
gctggagccttgtacaccaatggcctg

SEQ ID NO: 113 - DNA, 29 bp, synthetic construct
  source 1..29: mol_type = other DNA; note = ND1-C-D450A_R
gtacaaggctccagctggcttgcgagatc

SEQ ID NO: 114 - DNA, 29 bp, synthetic construct
  source 1..29: mol_type = other DNA; note = ND1-C-D467A_F
gctacgaaagcgtataaggacggctatag

SEQ ID NO: 115 - DNA, 27 bp, synthetic construct
  source 1..27: mol_type = other DNA; note = ND1-C-D467A_R
atacgctttcgtagccaggataatgcc

SEQ ID NO: 116 - DNA, 18 bp, synthetic construct
  source 1..18: mol_type = other DNA; note = APC-R
tacagaagcgggcaaagn

SEQ ID NO: 117 - DNA, 18 bp, synthetic construct
  source 1..18: mol_type = other DNA; note = APC-L
tatgtacgcctccctggn

SEQ ID NO: 118 - DNA, 20 bp, synthetic construct
  source 1..20: mol_type = other DNA; note = APC-L2-1
tcggcgccccctatgtacgn

SEQ ID NO: 119 - DNA, 21 bp, synthetic construct
  source 1..21: mol_type = other DNA; note = APC-L2-2
tcggcgccccctatgtacgcn

SEQ ID NO: 120 - DNA, 22 bp, synthetic construct
  source 1..22: mol_type = other DNA; note = APC-L2-3
tcggcgccccctatgtacgccn

SEQ ID NO: 121 - DNA, 17 bp, synthetic construct
  source 1..17: mol_type = other DNA; note = Rosa26-L
tgcccagaagactcccn

SEQ ID NO: 122 - DNA, 18 bp, synthetic construct
  source 1..18: mol_type = other DNA; note = Rosa26-R
tgatctgcaagtcgaggn

SEQ ID NO: 123 - DNA, 19 bp, synthetic construct
  source 1..19: mol_type = other DNA; note = Rosa26-LM4.2
tcctgacccctcccgggan

SEQ ID NO: 124 - DNA, 18 bp, synthetic construct
  source 1..18: mol_type = other DNA; note = Rosa26-LM3.2
tcctgacccctcccgggn

SEQ ID NO: 125 - DNA, 17 bp, synthetic construct
  source 1..17: mol_type = other DNA; note = Rosa26-LM2.2
tcctgacccctcccggn

SEQ ID NO: 126 - DNA, 18 bp, synthetic construct
  source 1..18: mol_type = other DNA; note = Rosa26-LM1.2
tgtcctgacccctcccgn

SEQ ID NO: 127 - DNA, 17 bp, synthetic construct
  source 1..17: mol_type = other DNA; note = Rosa26-LM.2
tgtcctgacccctcccn

SEQ ID NO: 128 - DNA, 20 bp, synthetic construct
  source 1..20: mol_type = other DNA; note = Rosa26-LM.2+1
tccgtgtcctgacccctccn

SEQ ID NO: 129 - DNA, 19 bp, synthetic construct
  source 1..19: mol_type = other DNA; note = Rosa26-LM.2+2
tccgtgtcctgacccctcn

SEQ ID NO: 130 - DNA, 18 bp, synthetic construct
  source 1..18: mol_type = other DNA; note = Rosa26-LM.2+3
tccgtgtcctgacccctn

SEQ ID NO: 131 - DNA, 17 bp, synthetic construct
  source 1..17: mol_type = other DNA; note = Rosa26-LM.2+4
tccgtgtcctgaccccn

SEQ ID NO: 132 - DNA, 18 bp, synthetic construct
  source 1..18: mol_type = other DNA; note = HPRT1-R
tcgacatagtgattaggn

SEQ ID NO: 133 - DNA, 18 bp, synthetic construct
  source 1..18: mol_type = other DNA; note = HPRT1-L
tgaaccaggctatgaccn

SEQ ID NO: 134 - DNA, 18 bp, synthetic construct
  source 1..18: mol_type = other DNA; note = Negative control TALE
ttgcgcgtatagtcgcgn

SEQ ID NO: 135 - DNA, 23 bp, synthetic construct
  source 1..23: mol_type = other DNA; note = Rosa26-gRNA-A
gcctcgacttgcagatcacgagg

SEQ ID NO: 136 - DNA, 23 bp, synthetic construct
  source 1..23: mol_type = other DNA; note = Rosa26-gRNA-B
tgagggctaacctggtgcgtggg

SEQ ID NO: 137 - DNA, 23 bp, synthetic construct
  source 1..23: mol_type = other DNA; note = Rosa26-gRNA-C
ggaagggatccttccagtcccgg

SEQ ID NO: 138 - DNA, 23 bp, synthetic construct
  source 1..23: mol_type = other DNA; note = Rosa26-gRNA-D
ggagatgggcgggagtcttctgg

SEQ ID NO: 139 - DNA, 23 bp, synthetic construct
  source 1..23: mol_type = other DNA; note = APC-gRNA-A
tctgtaccaccctcagttctcgg

SEQ ID NO: 140 - DNA, 23 bp, synthetic construct
  source 1..23: mol_type = other DNA; note = APC-gRNA-B
gggggcgccgaggcccgagaagg

SEQ ID NO: 141 - DNA, 23 bp, synthetic construct
  source 1..23: mol_type = other DNA; note = APC-gRNA-C
gttctcgggtcctggagcaccgg

SEQ ID NO: 142 - DNA, 23 bp, synthetic construct
  source 1..23: mol_type = other DNA; note = APC-gRNA-D
cccagggaggcgtacataggggg

SEQ ID NO: 143 - DNA, 23 bp, synthetic construct
  source 1..23: mol_type = other DNA; note = HPRT1-gRNA-A
taatcactatgtcgaggatttgg

SEQ ID NO: 144 - DNA, 23 bp, synthetic construct
  source 1..23: mol_type = other DNA; note = HPRT1-gRNA-B
aataagccttagttcgccagagg

SEQ ID NO: 145 - DNA, 23 bp, synthetic construct
  source 1..23: mol_type = other DNA; note = HPRT1-gRNA-C
gaaaaggtgtttattcctcatgg

SEQ ID NO: 146 - DNA, 23 bp, synthetic construct
  source 1..23: mol_type = other DNA; note = HPRT1-gRNA-D
aataaatctaggtcatagcctgg

SEQ ID NO: 147 - DNA, 23 bp, synthetic construct
  source 1..23: mol_type = other DNA; note = gRNA-off4-L3
ggggaaattgagtttcggccagg

SEQ ID NO: 148 - DNA, 23 bp, synthetic construct
  source 1..23: mol_type = other DNA; note = gRNA-off4-L4
ggccgaaactcaatttcccctgg

SEQ ID NO: 149 - DNA, 23 bp, synthetic construct
  source 1..23: mol_type = other DNA; note = gRNA-off4-L5
tcaatttcccctggtagaaatgg

SEQ ID NO: 150 - DNA, 23 bp, synthetic construct
  source 1..23: mol_type = other DNA; note = gRNA-CBE-L4M2
agacggatatctcccgggagggg

SEQ ID NO: 151 - DNA, 23 bp, synthetic construct
  source 1..23: mol_type = other DNA; note = gRNA-ABE-L4M2
gcttagtctatctcccgggaggg

SEQ ID NO: 152 - DNA, 62 bp, synthetic construct
  source 1..62: mol_type = other DNA; note = Rosa26-L2
ctagctacagaagcgggcaaaggctatttgggaagacggatcgggagtcttctgggcacggc

SEQ ID NO: 153 - DNA, 65 bp, synthetic construct
  source 1..65: mol_type = other DNA; note = Rosa26-L3
ctagctacagaagcgggcaaaggctatttgggaagacggatatccgggagtcttctgggcacggc

SEQ ID NO: 154 - DNA, 68 bp, synthetic construct
  source 1..68: mol_type = other DNA; note = Rosa26-L4
ctagctacagaagcgggcaaaggctatttgggaagacggatatctcccgggagtcttctgggcacggc

SEQ ID NO: 155 - DNA, 71 bp, synthetic construct
  source 1..71: mol_type = other DNA; note = Rosa26-L5
ctagctacagaagcgggcaaaggctatttgggaagacggatatctcctgccgggagtcttctgggcacggc

SEQ ID NO: 156 - DNA, 74 bp, synthetic construct
  source 1..74: mol_type = other DNA; note = Rosa26-R1
ctagctacagaagcgggcaaaggctatttgggaagacggatatctcctgcaggcgggagtcttctgggcacggc

SEQ ID NO: 157 - DNA, 65 bp, synthetic construct
  source 1..65: mol_type = other DNA; note = CBE-L4M2-7bp
ctagctacagaagcgggcaaagggggaagacggatatctcccgggaggggtcaggacacggaggc

SEQ ID NO: 158 - DNA, 66 bp, synthetic construct
  source 1..66: mol_type = other DNA; note = CBE-L4M2-8bp
ctagctacagaagcgggcaaaggtgggaagacggatatctcccgggaggggtcaggacacggaggc

SEQ ID NO: 159 - DNA, 67 bp, synthetic construct
  source 1..67: mol_type = other DNA; note = CBE-L4M2-9bp
ctagctacagaagcgggcaaaggttgggaagacggatatctcccgggaggggtcaggacacggaggc

SEQ ID NO: 160 - DNA, 68 bp, synthetic construct
  source 1..68: mol_type = other DNA; note = CBE-L4M2-10bp
ctagctacagaagcgggcaaaggtttgggaagacggatatctcccgggaggggtcaggacacggaggc

SEQ ID NO: 161 - DNA, 69 bp, synthetic construct
  source 1..69: mol_type = other DNA; note = CBE-L4M2-11bp
ctagctacagaagcgggcaaaggatttgggaagacggatatctcccgggaggggtcaggacacggaggc

SEQ ID NO: 162 - DNA, 70 bp, synthetic construct
  source 1..70: mol_type = other DNA; note = CBE-L4M2-12bp
ctagctacagaagcgggcaaaggtatttgggaagacggatatctcccgggaggggtcaggacacggaggc

SEQ ID NO: 163 - DNA, 71 bp, synthetic construct
  source 1..71: mol_type = other DNA; note = CBE-L4M2-13bp
ctagctacagaagcgggcaaaggctatttgggaagacggatatctcccgggaggggtcaggacacggaggc

SEQ ID NO: 164 - DNA, 72 bp, synthetic construct
  source 1..72: mol_type = other DNA; note = CBE-L4M2-14bp
ctagctacagaagcgggcaaaggtctatttgggaagacggatatctcccgggaggggtcaggacacggaggc

SEQ ID NO: 165 - DNA, 73 bp, synthetic construct
  source 1..73: mol_type = other DNA; note = CBE-L4M2-15bp
ctagctacagaagcgggcaaagggtctatttgggaagacggatatctcccgggaggggtcaggacacggaggc

SEQ ID NO: 166 - DNA, 74 bp, synthetic construct
  source 1..74: mol_type = other DNA; note = CBE-L4M2-16bp
ctagctacagaagcgggcaaaggagtctatttgggaagacggatatctcccgggaggggtcaggacacggaggc

SEQ ID NO: 167 - DNA, 65 bp, synthetic construct
  source 1..65: mol_type = other DNA; note = ABE-L4M2-7bp
ctagccctttgcccgcttctgtaatggcttagtctatctcccgggaggggtcaggacacggaggc

SEQ ID NO: 168 - DNA, 66 bp, synthetic construct
  source 1..66: mol_type = other DNA; note = ABE-L4M2-8bp
ctagccctttgcccgcttctgtaaatggcttagtctatctcccgggaggggtcaggacacggaggc

SEQ ID NO: 169 - DNA, 67 bp, synthetic construct
  source 1..67: mol_type = other DNA; note = ABE-L4M2-9bp
ctagccctttgcccgcttctgtaacatggcttagtctatctcccgggaggggtcaggacacggaggc

SEQ ID NO: 170 - DNA, 68 bp, synthetic construct
  source 1..68: mol_type = other DNA; note = ABE-L4M2-10bp
ctagccctttgcccgcttctgtaaacatggcttagtctatctcccgggaggggtcaggacacggaggc

SEQ ID NO: 171 - DNA, 69 bp, synthetic construct
  source 1..69: mol_type = other DNA; note = ABE-L4M2-11bp
ctagccctttgcccgcttctgtacaacatggcttagtctatctcccgggaggggtcaggacacggaggc

SEQ ID NO: 172 - DNA, 70 bp, synthetic construct
  source 1..70: mol_type = other DNA; note = ABE-L4M2-12bp
ctagccctttgcccgcttctgtaacatgcgcgcttagtctatctcccgggaggggtcaggacacggaggc

SEQ ID NO: 173 - DNA, 71 bp, synthetic construct
  source 1..71: mol_type = other DNA; note = ABE-L4M2-13bp
ctagccctttgcccgcttctgtaaacatgcgcgcttagtctatctcccgggaggggtcaggacacggaggc

SEQ ID NO: 174 - DNA, 72 bp, synthetic construct
  source 1..72: mol_type = other DNA; note = ABE-L4M2-14bp
ctagccctttgcccgcttctgtacaacatgcgcgcttagtctatctcccgggaggggtcaggacacggaggc

SEQ ID NO: 175 - DNA, 73 bp, synthetic construct
  source 1..73: mol_type = other DNA; note = ABE-L4M2-15bp
ctagccctttgcccgcttctgtaccaacatgcgcgcttagtctatctcccgggaggggtcaggacacggaggc

SEQ ID NO: 176 - DNA, 74 bp, synthetic construct
  source 1..74: mol_type = other DNA; note = ABE-L4M2-16bp
ctagccctttgcccgcttctgtacccaacatgcgcgcttagtctatctcccgggaggggtcaggacacggaggc

SEQ ID NO: 177 - DNA, 30 bp, synthetic construct
  source 1..30: mol_type = other DNA; note = APC-F2
catgcgcattgtagtcttcccacctcccac

SEQ ID NO: 178 - DNA, 26 bp, synthetic construct
  source 1..26: mol_type = other DNA; note = APC-R
cgtctggcaggtgagtgaggctgcag

SEQ ID NO: 179 - DNA, 28 bp, synthetic construct
  source 1..28: mol_type = other DNA; note = off4-F
agtcctgtttctaaaaaaggcccacccc

SEQ ID NO: 180 - DNA, 27 bp, synthetic construct
  source 1..27: mol_type = other DNA; note = off4-R
gttctgttggctcatctgtctacctgg

SEQ ID NO: 181 - DNA, 18 bp, synthetic construct
  source 1..18: mol_type = other DNA; note = off4-L
tgcccagcaaccattaan

SEQ ID NO: 182 - DNA, 72 bp, synthetic construct
  source 1..72: mol_type = other DNA; note = APC-site1
ggtggtacagaagcgggcaaaggggcgaccggacccgagcccagggaggcgtacatagggggcgccgaggcc

SEQ ID NO: 183 - protein, 4 aa, synthetic construct
SAGG

SEQ ID NO: 184 - protein, 16 aa, synthetic construct
SGSETPGTSESATPES

SEQ ID NO: 185 - DNA, 44 bp, synthetic construct
  source 1..44: mol_type = other DNA
gccacccctgaatcctctgaggtggagttttcccacgagtattg

SEQ ID NO: 186 - DNA, 42 bp, synthetic construct
  source 1..42: mol_type = other DNA
cactgtgctggattagttgatggagctctgggccttcttctg

SEQ ID NO: 187 - DNA, 29 bp, synthetic construct
  source 1..29: mol_type = other DNA
tctgaggtggagttttcccacgagtattg

SEQ ID NO: 188 - DNA, 38 bp, synthetic construct
  source 1..38: mol_type = other DNA
agagccgctgactaggagtgcggccagcgcggggtccg

SEQ ID NO: 189 - DNA, 26 bp, synthetic construct
  source 1..26: mol_type = other DNA
taatccagcacagtggcggccgctcg

SEQ ID NO: 190 - DNA, 39 bp, synthetic construct
  source 1..39: mol_type = other DNA
agagccgctgactagggatctgatcaattccggcgcgtg

SEQ ID NO: 191 - DNA, 39 bp, synthetic construct
  source 1..39: mol_type = other DNA
aaactccacctcagaggatctgatcaattccggcgcgtg

SEQ ID NO: 192 - DNA, 40 bp, synthetic construct
  source 1..40: mol_type = other DNA
aaactccacctcagagctggcctccacctttctcttcttc

SEQ ID NO: 193 - DNA, 498 bp, synthetic construct
  source 1..498: mol_type = other DNA
tctgaggtggagttttcccacgagtattggatgagacatgcactgaccctggcaaagagggcacgcgatgagagggaagtccctgtcggcgccgtgctggtgctgaacaacagagtgatcggcgagggatggaacagggcaatcggcctgcacgaccctacagcccatgccgaaattatggccctgaggcagggaggcctggtcatgcagaactaccgcctgattgacgccaccctgtacgtgacattcgagccttgcgtgatgtgcgccggcgcaatgatccacagcaggatcggaagggtggtgtttggctggcgcaactcaaaaagaggagcagcaggctccctgatgaacgtgctgaactacccaggcatgaatcaccgggtcgaaattaccgagggaatcctggcagatgaatgtgccgccctgctgtgcgatttctatcggatgcccagacaggtgttcaatgctcagaagaaggcccagagctccatcaac

SEQ ID NO: 194 - protein, 166 aa, synthetic construct
SEVEFSHEYWMRHALTLAKRARDEREVPVGAVLVLNNRVIGEGWNRAIGLHDPTAHAEIMALRQGGLVMQNYRLIDATLYVTFEPCVMCAGAMIHSRIGRVVFGWRNSKRGAAGSLMNVLNYPGMNHRVEITEGILADECAALLCDFYRMPRQVFNAQKKAQSSIN

SEQ ID NO: 195 - DNA, 671 bp, synthetic construct
  source 1..671: mol_type = other DNA
atggcttcctcccctccaaagaaaaagagaaaggttgcggccgctgactacaaggatgacgacgataaaagttggaaggacgcaagtggttggtctagaatgcatgcggccccgcgacggcgtgctgcgcaaccctccgacgcttcgccggccgcgcaggtggatctacgcacgctcggctacagtcagcagcagcaagagaagatcaaaccgaaggtgcgttcgacagtggcgcagcaccacgaggcactggtgggccatgggtttacacacgcgcacatcgttgcgctcagccaacacccggcagcgttagggaccgtcgctgtcacgtatcagcacataatcacggcgttgccagaggcgacacacgaagacatcgttggcgtcggcaaacagtggtccggcgcacgcgccctggaggccttgctcacggatgcgggggagttgagaggtccgccgttacagttggacacaggccaacttgtgaagattgcaaaacgtggcggcgtgaccgcaatggaggcagtgcatgcatcgcgcaatgcgctcacgggagcacccctcaagacccctgagcaggtagtggctattgcatccaacaacgggggcagacccgcactggagtcaatcgtggcccagctttcgaggccggaccccgcgctggccgcact

SEQ ID NO: 196 - protein, 224 aa, synthetic construct
MASSPPKKKRKVAAADYKDDDDKSWKDASGWSRMHAAPRRRAAQPSDASPAAQVDLRTLGYSQQQQEKIKPKVRSTVAQHHEALVGHGFTHAHIVALSQHPAALGTVAVTYQHIITALPEATHEDIVGVGKQWSGARALEALLTDAGELRGPPLQLDTGQLVKIAKRGGVTAMEAVHASRNALTGAPLKTPEQVVAIASNNGGRPALESIVAQLSRPDPALAAL

SEQ ID NO: 197 - DNA, 56 bp, synthetic construct
  source 1..56: mol_type = other DNA
ctagtcagcggctctgagacccccggaacaagcgaatctgccacccctgaatccgg

SEQ ID NO: 198 - protein, 18 aa, synthetic construct
LVSGSETPGTSESATPES

SEQ ID NO: 199 - DNA, 672 bp, synthetic construct
  source 1..672: mol_type = other DNA
cccagacagctggaagaagtgatcgatctgctggaagtgtaccacgagaagaaaaacgtgatcgaggaaaagattaaggcccggtttatcgccaacaagaacaccgtgttcgagtggctgacctggaacggcttcatcatcctgggcaacgccctcgagtacaagaacaacttcgtgatcgatgaggaactgcagcccgtgacacacgccgctggaaaccagcctgacatggaaatcatctacgaggacttcatcgtgctgggcgaagtgaccacaagcaagggcgccacacagttcaagatggaaagcgagcctgtgaccagacactacctcaacaaaaagaaagagctggaaaagcagggcgtcgagaaagaactgtactgcctgttcattgcccctgagatcaacaagaataccttcgaggaattcatgaagtacaacatcgtgcagaacacccggatcatccctctgtctctgaagcagttcaacatgctgctcatggtgcagaagaaactcatcgagaaaggcagacggctgagcagctacgacatcaagaacctgatggtgtccctgtaccggaccaccatcgagtgcgagagaaagtacacccagatcaaggccggactggaagagacactgaacaactgggtcgtcgacaaagaagtgcggttc

SEQ ID NO: 200 - protein, 224 aa, synthetic construct
PRQLEEVIDLLEVYHEKKNVIEEKIKARFIANKNTVFEWLTWNGFIILGNALEYKNNFVIDEELQPVTHAAGNQPDMEIIYEDFIVLGEVTTSKGATQFKMESEPVTRHYLNKKKELEKQGVEKELYCLFIAPEINKNTFEEFMKYNIVQNTRIIPLSLKQFNMLLMVQKKLIEKGRRLSSYDIKNLMVSLYRTTIECERKYTQIKAGLEETLNNWVVDKEVRF

SEQ ID NO: 201 - DNA, 42 bp, synthetic construct
  source 1..42: mol_type = other DNA
aggccggaccccgcgagacagctggaagaagtgatcgatctg

SEQ ID NO: 202 - DNA, 43 bp, synthetic construct
  source 1..43: mol_type = other DNA
cgccactgtgctggattagaaccgcacttctttgtcgacgacc

SEQ ID NO: 203 - DNA, 28 bp, synthetic construct
  source 1..28: mol_type = other DNA
cgcggggtccggcctcgaaagctgggcc

SEQ ID NO: 204 - DNA, 27 bp, synthetic construct
  source 1..27: mol_type = other DNA
tccagcacagtggcggccgctcgagtc

SEQ ID NO: 205 - DNA, 723 bp, synthetic construct
  source 1..723: mol_type = other DNA
atggactataaggaccacgacggagactacaaggatcatgatattgattacaaagacgatgacgataagatggccccaaagaagaagcggaaggtcggtatccacggagtcccagcagccatggacatcgccgatttgagaactttgggatattcacagcagcagcaggaaaagatcaagcccaaagtgaggtcgacagtcgcgcagcatcacgaagcgctggtgggtcatgggtttacacatgcccacatcgtagccttgtcgcagcaccctgcagcccttggcacggtcgccgtcaagtaccaggacatgattgcggcgttgccggaagccacacatgaggcgatcgtcggtgtggggaaacagtggagcggagcccgagcgcttgaggccctgttgacggtcgcgggagagctgagagggcctccccttcagctggacacgggccagttgctgaagatcgcgaagcggggaggagtcacggcggtcgaggcggtacacgcgtggcgcaatgcgctcacgggagcacccctcaagacccctgagcaggtagtggctattgcatccaacaacgggggcaaacaggcactggagtcaatcgtggcccagctttcgaggccggaccccgcgctggccgcactcactaatgatcatcttgtagcgctggcctgcctcggcggacgtcctgccctggatgcagtgaaaaagggattgggaggcagc

SEQ ID NO: 206 - protein, 241 aa, synthetic construct
MDYKDHDGDYKDHDIDYKDDDDKMAPKKKRKVGIHGVPAAMDIADLRTLGYSQQQQEKIKPKVRSTVAQHHEALVGHGFTHAHIVALSQHPAALGTVAVKYQDMIAALPEATHEAIVGVGKQWSGARALEALLTVAGELRGPPLQLDTGQLLKIAKRGGVTAVEAVHAWRNALTGAPLKTPEQVVAIASNNGGKQALESIVAQLSRPDPALAALTNDHLVALACLGGRPALDAVKKGLGGS

SEQ ID NO: 207 - DNA, 36 bp, synthetic construct
  source 1..36: mol_type = other DNA
ggaggcagcagacagctggaagaagtgatcgatctg

SEQ ID NO: 208 - DNA, 52 bp, synthetic construct
  source 1..52: mol_type = other DNA
ctgtctgctgcctcccaatccctttttcactgcatccagggcaggacgtccg

SEQ ID NO: 209 - DNA, 43 bp, synthetic construct
  source 1..43: mol_type = other DNA
atcggcgatgtccatggctgctgggactccgtggataccgacc

SEQ ID NO: 210 - DNA, 40 bp, synthetic construct
  source 1..40: mol_type = other DNA
atggacatcgccgatttgagaactttgggatattcacagc

SEQ ID NO: 211 - DNA, 33 bp, synthetic construct
  source 1..33: mol_type = other DNA
ctgtttgcccccgttgttggatgcaatagccac

SEQ ID NO: 212 - DNA, 45 bp, synthetic construct
  source 1..45: mol_type = other DNA
caacgggggcaaacaggcactggagtcaatcgtggcccagctttc

SEQ ID NO: 213 - DNA, 44 bp, synthetic construct
  source 1..44: mol_type = other DNA
cttaaggccaccatggcccttagccgagctgtgtgtggcacctc

SEQ ID NO: 214 - DNA, 40 bp, synthetic construct
  source 1..40: mol_type = other DNA
atcggcgatgtccatcttgtcgtcatcatccttatagtcg

SEQ ID NO: 215 - DNA, 40 bp, synthetic construct
  source 1..40: mol_type = other DNA
ggcggcgatgtccatcttgtcgtcatcatccttatagtcg

SEQ ID NO: 216 - DNA, 39 bp, synthetic construct
  source 1..39: mol_type = other DNA
cttaaggccaccatggcctctgtcctgacacctctgctg

SEQ ID NO: 217 - DNA, 40 bp, synthetic construct
  source 1..40: mol_type = other DNA
ggcggcgatgtccatggcgtaatcgggcacgtcatatggg

SEQ ID NO: 218 - DNA, 37 bp, synthetic construct
  source 1..37: mol_type = other DNA
atggacatcgccgccccgcgacggcgtgctgcgcaac

SEQ ID NO: 219 - DNA, 27 bp, synthetic construct
  source 1..27: mol_type = other DNA
catggtggccttaagtttaaacgctag

SEQ ID NO: 220 - DNA, 189 bp, synthetic construct
  source 1..189: mol_type = other DNA
atggcctctgtcctgacacctctgctgcttcgtgggttgactggaagtgcacgcaggctgcctgtacctagagccaagattcactccctgtatccgtacgatgtcccggactatgcaggctatccctacgatgtacccgattatgccggatacccatatgacgtgcccgattacgccatggacatcgcc

SEQ ID NO: 221 - protein, 63 aa, synthetic construct
MASVLTPLLLRGLTGSARRLPVPRAKIHSLYPYDVPDYAGYPYDVPDYAGYPYDVPDYAMDIA

SEQ ID NO: 222 - DNA, 171 bp, synthetic construct
  source 1..171: mol_type = other DNA
atggcccttagccgagctgtgtgtggcacctcaaggcaactggccccagtgctggggtacttggggtcacggcagaagcactcactgcctgatgattacaaggaccatgacggagactacaaagaccatgacatcgactataaggatgatgacgacaagatggacatcgcc

SEQ ID NO: 223 - protein, 57 aa, synthetic construct
MALSRAVCGTSRQLAPVLGYLGSRQKHSLPDDYKDHDGDYKDHDIDYKDDDDKMDIA

SEQ ID NO: 224 - DNA, 19 bp, synthetic construct
  source 1..19: mol_type = other DNA
tgagtttgatgctcacccn

SEQ ID NO: 225 - DNA, 18 bp, synthetic construct
  source 1..18: mol_type = other DNA
tagccacctctagcctan

SEQ ID NO: 226 - DNA, 16 bp, synthetic construct
  source 1..16: mol_type = other DNA
tctagcctagccgttn

SEQ ID NO: 227 - DNA, 21 bp, synthetic construct
  source 1..21: mol_type = other DNA
aatatgattagttctgtggcn

SEQ ID NO: 228 - DNA, 18 bp, synthetic construct
  source 1..18: mol_type = other DNA
tactaatctccctacaan

SEQ ID NO: 229 - DNA, 21 bp, synthetic construct
  source 1..21: mol_type = other DNA
aatctccctacaaatctcctn

SEQ ID NO: 230 - DNA, 20 bp, synthetic construct
  source 1..20: mol_type = other DNA
tgcttattgctgaggggcan

SEQ ID NO: 231 - DNA, 20 bp, synthetic construct
  source 1..20: mol_type = other DNA
tccatgctgtcaagcccagn

SEQ ID NO: 232 - DNA, 19 bp, synthetic construct
  source 1..19: mol_type = other DNA
tgtcaagcccagcagtctn

SEQ ID NO: 233 - DNA, 20 bp, synthetic construct
  source 1..20: mol_type = other DNA
tctagtgcaagctaacagtn

SEQ ID NO: 234 - DNA, 21 bp, synthetic construct
  source 1..21: mol_type = other DNA
taatcagaggccaaacccttn

SEQ ID NO: 235 - DNA, 22 bp, synthetic construct
  source 1..22: mol_type = other DNA
tcagaggccaaacccttcctgn

SEQ ID NO: 236 - DNA, 19 bp, synthetic construct
  source 1..19: mol_type = other DNA
ttctcgcggctccgctcgn

SEQ ID NO: 237 - DNA, 20 bp, synthetic construct
  source 1..20: mol_type = other DNA
tcgcttcggaggagccgtgn

SEQ ID NO: 238 - DNA, 20 bp, synthetic construct
  source 1..20: mol_type = other DNA
tcggaggagccgtggtccgn

SEQ ID NO: 239 - DNA, 21 bp, synthetic construct
  source 1..21: mol_type = other DNA
tccagccctggcctgggtcan

SEQ ID NO: 240 - DNA, 18 bp, synthetic construct
  source 1..18: mol_type = other DNA
tcctctgccatcacgtgn

SEQ ID NO: 241 - DNA, 22 bp, synthetic construct
  source 1..22: mol_type = other DNA
tcctctgccatcacgtgctcan

SEQ ID NO: 242 - DNA, 26 bp, synthetic construct
  source 1..26: mol_type = other DNA
gctctcaccatcgctcttctactatg

SEQ ID NO: 243 - DNA, 27 bp, synthetic construct
  source 1..27: mol_type = other DNA
atgatggctagggtgacttcatatgag

SEQ ID NO: 244 - DNA, 24 bp, synthetic construct
  source 1..24: mol_type = other DNA
catggcaagccaacgccacttatc

SEQ ID NO: 245 - DNA, 28 bp, synthetic construct
  source 1..28: mol_type = other DNA
gtgagtgtaaattagtgcgatgagtagg

SEQ ID NO: 246 - DNA, 215 bp, synthetic construct
  source 1..215: mol_type = other DNA
gctctcaccatcgctcttctactatgaacccccctccccatacccaaccccctggtcaacctcaacctaggcctcctatttattctagccacctctagcctagccgtttactcaatcctctgatcagggtgagcatcaaactcaaactacgccctgatcggcgcactgcgagcagtagcccaaacaatctcatatgaagtcaccctagccatcat

SEQ ID NO: 247 - DNA, 274 bp, synthetic construct
  source 1..274: mol_type = other DNA
catggcaagccaacgccacttatccagtgaaccactatcacgaaaaaaactctacctctctatactaatctccctacaaatctccttaattataacattcacagccacagaactaatcatattttatatcttcttcgaaaccacacttatccccaccttggctatcatcacccgatgaggcaaccagccagaacgcctgaacgcaggcacatacttcctattctacaccctagtaggctcccttcccctactcatcgcactaatttacactcac

SEQ ID NO: 248 - DNA, 415 bp, synthetic construct
  source 1..415: mol_type = other DNA
gagcccctaaaacccgccacatctaccatcaccctctacatcaccgccccgaccttagctctcaccatcgctcttctactatgaacccccctccccatacccaaccccctggtcaacctcaacctaggcctcctatttattctagccacctctagcctagccgtttactcaatcctctgatcagggtgagcatcaaactcaaactacgccctgatcggcgcactgcgagcagtagcccaaacaatctcatatgaagtcaccctagccatcattctactatcaacattactaataagtggctcctttaacctctccacccttatcacaacacaagaacacctctgattactcctgccatcatgacccttggccataatatgatttatctccacactagcagagaccaaccgaaccc

SEQ ID NO: 249 - DNA, 616 bp, synthetic construct
  source 1..616: mol_type = other DNA
caatctccaacacatatggcctagactacgtacataacctaaacctactccaatgctaaaactaatcgtcccaacaattatattactaccactgacatgactttccaaaaaacacataatttgaatcaacacaaccacccacagcctaattattagcatcatccctctactattttttaaccaaatcaacaacaacctatttagctgttccccaaccttttcctccgaccccctaacaacccccctcctaatactaactacctgactcctacccctcacaatcatggcaagccaacgccacttatccagtgaaccactatcacgaaaaaaactctacctctctatactaatctccctacaaatctccttaattataacattcacagccacagaactaatcatattttatatcttcttcgaaaccacacttatccccaccttggctatcatcacccgatgaggcaaccagccagaacgcctgaacgcaggcacatacttcctattctacaccctagtaggctcccttcccctactcatcgcactaatttacactcacaacaccctaggctcactaaacattctactactcactctcactgcccaagaactatcaaac

SEQ ID NO: 250 - DNA, 25 bp, synthetic construct
  source 1..25: mol_type = other DNA
cagggttttcccagtcacgacgttg

SEQ ID NO: 251 - DNA, 25 bp, synthetic construct
  source 1..25: mol_type = other DNA
cacgacaggtttcccgactggaaag

SEQ ID NO: 252 - DNA, 27 bp, synthetic construct
  source 1..27: mol_type = other DNA
gagcccctaaaacccgccacatctacc

SEQ ID NO: 253 - DNA, 26 bp, synthetic construct
  source 1..26: mol_type = other DNA
gggttcggttggtctctgctagtgtg

SEQ ID NO: 254 - DNA, 26 bp, synthetic construct
  source 1..26: mol_type = other DNA
caatctccaacacatatggcctagac

SEQ ID NO: 255 - DNA, 26 bp, synthetic construct
  source 1..26: mol_type = other DNA
gtttgatagttcttgggcagtgagag

SEQ ID NO: 256 - DNA, 28 bp, synthetic construct
  source 1..28: mol_type = other DNA
ctcactcattaggcaccccaggctttac

SEQ ID NO: 257 - DNA, 27 bp, synthetic construct
  source 1..27: mol_type = other DNA
agaatgtttagtgagcctagggtgttg

SEQ ID NO: 258 - DNA, 29 bp, synthetic construct
  source 1..29: mol_type = other DNA
gctagaaggagaggccagttaagacagtg

SEQ ID NO: 259 - DNA, 27 bp, synthetic construct
  source 1..27: mol_type = other DNA
cctgacaaagctcagctcctctcctag

SEQ ID NO: 260 - DNA, 28 bp, synthetic construct
  source 1..28: mol_type = other DNA
gtgagatggctgaaaagcgatacagggc

SEQ ID NO: 261 - DNA, 27 bp, synthetic construct
  source 1..27: mol_type = other DNA
gccaccgatggagaggtctgccagtcc

SEQ ID NO: 262 - DNA, 26 bp, synthetic construct
  source 1..26: mol_type = other DNA
gcggcggcgagccgcgggcaggggcc

SEQ ID NO: 263 - DNA, 26 bp, synthetic construct
  source 1..26: mol_type = other DNA
ggctggagcactgtctgcgcacaccg

SEQ ID NO: 264 - DNA, 27 bp, synthetic construct
  source 1..27: mol_type = other DNA
tcctgcagggagcttggcatgagaaac

SEQ ID NO: 265 - DNA, 27 bp, synthetic construct
  source 1..27: mol_type = other DNA
tgtcaaccagtatcccggtgcaggagc

SEQ ID NO: 266 - DNA, 23 bp, synthetic construct
  source 1..23: mol_type = other DNA
agtgaagaccaaggatagactgc

SEQ ID NO: 267 - DNA, 23 bp, synthetic construct
  source 1..23: mol_type = other DNA
gcttttatcacaggctccaggaa

SEQ ID NO: 268 - DNA, 20 bp, synthetic construct
  source 1..20: mol_type = other DNA
ctcggcttcccccgcgcgga

SEQ ID NO: 269 - DNA, 30 bp, synthetic construct
  source 1..30: mol_type = other DNA
tccttggggcccagactgagcacgtgatgg

SEQ ID NO: 270 - DNA, 20 bp, synthetic construct
  source 1..20: mol_type = other DNA
tacccagaaccagagccaca

SEQ ID NO: 271 - DNA, 20 bp, synthetic construct
  source 1..20: mol_type = other DNA
tgttttgtctgagggtgagg

SEQ ID NO: 272 - DNA, 21 bp, synthetic construct
  source 1..21: mol_type = other DNA
tacagaagcgggcaaaggggc

SEQ ID NO: 273 - DNA, 21 bp, synthetic construct
  source 1..21: mol_type = other DNA
tcccatcaccatcaccaccac

SEQ ID NO: 274 - DNA, 20 bp, synthetic construct
  source 1..20: mol_type = other DNA
tccagcccgctggccctgta

SEQ ID NO: 275 - DNA, 19 bp, synthetic construct
  source 1..19: mol_type = other DNA
tggtattcttcagactata

SEQ ID NO: 276 - DNA, 19 bp, synthetic construct
  source 1..19: mol_type = other DNA
tgggtgggagtggcacttt

SEQ ID NO: 277 - DNA, 19 bp, synthetic construct
  source 1..19: mol_type = other DNA
ttcctttcctctgccatca

SEQ ID NO: 278 - DNA, 20 bp, synthetic construct
  source 1..20: mol_type = other DNA
ttcctttcctctgccatcac

SEQ ID NO: 279 - DNA, 21 bp, synthetic construct
  source 1..21: mol_type = other DNA
ttcctttcctctgccatcacg

SEQ ID NO: 280 - DNA, 22 bp, synthetic construct
  source 1..22: mol_type = other DNA
ttcctttcctctgccatcacgt

SEQ ID NO: 281 - DNA, 22 bp, synthetic construct
  source 1..22: mol_type = other DNA
tcctttcctctgccatcacgtg

SEQ ID NO: 282 - DNA, 19 bp, synthetic construct
  source 1..19: mol_type = other DNA
tcctctgccatcacgtgct

SEQ ID NO: 283 - DNA, 20 bp, synthetic construct
  source 1..20: mol_type = other DNA
tcctctgccatcacgtgctc

SEQ ID NO: 284 - DNA, 21 bp, synthetic construct
  source 1..21: mol_type = other DNA
tcctctgccatcacgtgctca

SEQ ID NO: 285 - DNA, 21 bp, synthetic construct
  source 1..21: mol_type = other DNA
tgttctcgcttcggaggagcc

SEQ ID NO: 286 - DNA, 20 bp, synthetic construct
  source 1..20: mol_type = other DNA
ttctcgcttcggaggagccg

SEQ ID NO: 287 - DNA, 21 bp, synthetic construct
  source 1..21: mol_type = other DNA
ttctcgcttcggaggagccgt

SEQ ID NO: 288 - DNA, 22 bp, synthetic construct
  source 1..22: mol_type = other DNA
ttctcgcttcggaggagccgtg

SEQ ID NO: 289 - DNA, 21 bp, synthetic construct
  source 1..21: mol_type = other DNA
tcgcttcggaggagccgtggt

SEQ ID NO: 290 - DNA, 18 bp, synthetic construct
  source 1..18: mol_type = other DNA
ttcggaggagccgtggtc

SEQ ID NO: 291 - DNA, 19 bp, synthetic construct
  source 1..19: mol_type = other DNA
ttcggaggagccgtggtcc

SEQ ID NO: 292 - DNA, 20 bp, synthetic construct
  source 1..20: mol_type = other DNA
ttcggaggagccgtggtccg

SEQ ID NO: 293 - DNA, 19 bp, synthetic construct
  source 1..19: mol_type = other DNA
taatcagaggccaaaccct

SEQ ID NO: 294 - DNA, 20 bp, synthetic construct
  source 1..20: mol_type = other DNA
taatcagaggccaaaccctt

SEQ ID NO: 295 - DNA, 19 bp, synthetic construct
  source 1..19: mol_type = other DNA
tcagaggccaaacccttcc

SEQ ID NO: 296 - DNA, 20 bp, synthetic construct
  source 1..20: mol_type = other DNA
tcagaggccaaacccttcct

SEQ ID NO: 297 - DNA, 21 bp, synthetic construct
  source 1..21: mol_type = other DNA
tcagaggccaaacccttcctg

SEQ ID NO: 298 - DNA, 19 bp, synthetic construct
  source 1..19: mol_type = other DNA
tccatgctgtcaagcccag

SEQ ID NO: 299 - DNA, 21 bp, synthetic construct
  source 1..21: mol_type = other DNA
tccatgctgtcaagcccagca

SEQ ID NO: 300 - DNA, 18 bp, synthetic construct
  source 1..18: mol_type = other DNA
tgctgtcaagcccagcag

SEQ ID NO: 301 - DNA, 19 bp, synthetic construct
  source 1..19: mol_type = other DNA
tgctgtcaagcccagcagt

SEQ ID NO: 302 - DNA, 20 bp, synthetic construct
  source 1..20: mol_type = other DNA
tgctgtcaagcccagcagtc

SEQ ID NO: 303 - DNA, 21 bp, synthetic construct
  source 1..21: mol_type = other DNA
tccccgagctgggaccacctt

SEQ ID NO: 304 - DNA, 22 bp, synthetic construct
  source 1..22: mol_type = other DNA
tcctcattttgtccactggtga

SEQ ID NO: 305 - DNA, 21 bp, synthetic construct
  source 1..21: mol_type = other DNA
tgggagataccccagtcagag

SEQ ID NO: 306 - DNA, 20 bp, synthetic construct
  source 1..20: mol_type = other DNA
tgttcatttccctgaagccc

SEQ ID NO: 307 - DNA, 19 bp, synthetic construct
  source 1..19: mol_type = other DNA
tgttcatttccctgaagcc

SEQ ID NO: 308 - DNA, 21 bp, synthetic construct
  source 1..21: mol_type = other DNA
ttacccaaggcttgttgtcca

SEQ ID NO: 309 - DNA, 20 bp, synthetic construct
  source 1..20: mol_type = other DNA
ttacccaaggcttgttgtcc

SEQ ID NO: 310 - DNA, 21 bp, synthetic construct
  source 1..21: mol_type = other DNA
tggcccgccccgcagtctatg

SEQ ID NO: 311 - DNA, 20 bp, synthetic construct
  source 1..20: mol_type = other DNA
tggcccgccccgcagtctat

SEQ ID NO: 312 - DNA, 1680 bp, synthetic construct
  source 1..1680: mol_type = other DNA
cccaagaagaagcggaaggtgagccctggcatccggagactggacgccctgatctctacaagcctgtacaagaaggccggctataaggaggcatccggatctggaagggcagacgcactggacgatttcgacctggatatgctgggctccgatgccctggacgattttgacctggacatgctgggatctgacgccctggatgactttgacctggatatgctgggaagtgacgctctggatgattttgacctggatatgctgatcaactccaggagctccggcagccccaagaagaagcggaaagtgggctctcagtacctgccagacacagacgatcggcacagaatcgaggagaagaggaagcgcacatatgagacattcaagtccatcatgaagaagagccccttttccggaccaaccgatcctcggccccctccaaggcgcatcgcagtgcctagcagatctagcgcctccgtgcctaagccagcaccacagccttaccccttcacctcctctctgtccaccatcaattatgacgagttccctaccatggtgtttccatctggacagatctctcaggcaagcgccctggcacctgccccccctcaggtgctgccacaggcaccagcacctgcaccagcaccagcaatggtgtccgccctggcccaggcccctgccccagtgcccgtgctggccccaggcccaccccaggcagtggcacctccagcacctaagccaacacaggcaggagagggcaccctgagcgaggccctgctgcagctgcagttcgacgatgaggacctgggcgccctgctgggaaactccacagatccagccgtgttcaccgacctggcaagcgtggataactccgagtttcagcagctgctgaatcagggcatcccagtggccccccacaccacagagccaatgctgatggagtaccccgaggccatcacacggctggtgaccggagcacagcggccccctgatccagcacctgccccactgggagcacctggcctgccaaatggcctgctgagcggcgacgaggatttcagctccatcgccgacatggatttttctgccctgctgggaagcggatccggctctagggacagccgcgagggcatgttcctgccaaagcctgaggcaggatccgccatctctgacgtgttcgagggaagggaggtgtgccagccaaagcggatcagacctttccacccaccaggctccccttgggcaaacaggccactgccagcctctctggcacctacaccaaccggaccagtgcacgagccagtgggcagcctgacaccagcacctgtgccacagcccctggaccctgccccagcagtgaccccagaggccagccacctgctggaggaccccgatgaggagacatcccaggcagtgaaggccctgagggagatggccgataccgtgatcccacagaaggaggaggcagcaatctgcggccagatggacctgtcccaccctccacccagaggccacctggatgagctgaccacaaccctggagtctatgaccgaggacctgaatctggatagccccctgacacctgagctgaacgagatcctggacacctttctgaatgatgagtgtctgctgcacgccatgcacatctctacaggcctgagcatcttcgacaccagcctgttt

SEQ ID NO: 313 - protein, 560 aa, synthetic construct
PKKKRKVSPGIRRLDALISTSLYKKAGYKEASGSGRADALDDFDLDMLGSDALDDFDLDMLGSDALDDFDLDMLGSDALDDFDLDMLINSRSSGSPKKKRKVGSQYLPDTDDRHRIEEKRKRTYETFKSIMKKSPFSGPTDPRPPPRRIAVPSRSSASVPKPAPQPYPFTSSLSTINYDEFPTMVFPSGQISQASALAPAPPQVLPQAPAPAPAPAMVSALAQAPAPVPVLAPGPPQAVAPPAPKPTQAGEGTLSEALLQLQFDDEDLGALLGNSTDPAVFTDLASVDNSEFQQLLNQGIPVAPHTTEPMLMEYPEAITRLVTGAQRPPDPAPAPLGAPGLPNGLLSGDEDFSSIADMDFSALLGSGSGSRDSREGMFLPKPEAGSAISDVFEGREVCQPKRIRPFHPPGSPWANRPLPASLAPTPTGPVHEPVGSLTPAPVPQPLDPAPAVTPEASHLLEDPDEETSQAVKALREMADTVIPQKEEAAICGQMDLSHPPPRGHLDELTTTLESMTEDLNLDSPLTPELNEILDTFLNDECLLHAMHISTGLSIFDTSLF

SEQ ID NO: 314 - DNA, 39 bp, synthetic construct
  source 1..39: mol_type = other DNA
gaattgatcagatcccccaagaagaagcggaaggtgagc

SEQ ID NO: 315 - DNA, 42 bp, synthetic construct
  source 1..42: mol_type = other DNA
cactgtgctggattaaaacaggctggtgtcgaagatgctcag

SEQ ID NO: 316 - DNA, 21 bp, synthetic construct
  source 1..21: mol_type = other DNA
tgaggaaggtgaagcactcag

SEQ ID NO: 317 - DNA, 21 bp, synthetic construct
  source 1..21: mol_type = other DNA
tactgttgttggctgttggtg

SEQ ID NO: 318 - DNA, 20 bp, synthetic construct
  source 1..20: mol_type = other DNA
tggctcgatgctgttcccag

SEQ ID NO: 319-329 - skipped (11 entries)

SEQ ID NO: 330 - DNA, 65 bp, synthetic construct
  source 1..65: mol_type = other DNA
ctagctacagaagcgggcaaaggatggcttagtctatctcccgggaggggtcaggacacggaggc

SEQ ID NO: 331 - DNA, 66 bp, synthetic construct
  source 1..66: mol_type = other DNA
ctagctacagaagcgggcaaagacatggcttagtctatctcccgggaggggtcaggacacggaggc

SEQ ID NO: 332 - DNA, 67 bp, synthetic construct
  source 1..67: mol_type = other DNA
ctagctacagaagcgggcaaagaacatggcttagtctatctcccgggaggggtcaggacacggaggc

SEQ ID NO: 333 - DNA, 68 bp, synthetic construct
  source 1..68: mol_type = other DNA
ctagctacagaagcgggcaaaggaacatggcttagtctatctcccgggaggggtcaggacacggaggc

SEQ ID NO: 334 - DNA, 69 bp, synthetic construct
  source 1..69: mol_type = other DNA
ctagctacagaagcgggcaaaggcaacatggcttagtctatctcccgggaggggtcaggacacggaggc

SEQ ID NO: 335 - DNA, 70 bp, synthetic construct
  source 1..70: mol_type = other DNA
ctagctacagaagcgggcaaagaacatgcgcgcttagtctatctcccgggaggggtcaggacacggaggc

SEQ ID NO: 336 - DNA, 71 bp, synthetic construct
  source 1..71: mol_type = other DNA
ctagctacagaagcgggcaaaggaacatgcgcgcttagtctatctcccgggaggggtcaggacacggaggc

SEQ ID NO: 337 - DNA, 72 bp, synthetic construct
  source 1..72: mol_type = other DNA
ctagctacagaagcgggcaaaggcaacatgcgcgcttagtctatctcccgggaggggtcaggacacggaggc

SEQ ID NO: 338 - DNA, 73 bp, synthetic construct
  source 1..73: mol_type = other DNA
ctagctacagaagcgggcaaaggccaacatgcgcgcttagtctatctcccgggaggggtcaggacacggaggc

SEQ ID NO: 339 - DNA, 74 bp, synthetic construct
  source 1..74: mol_type = other DNA
ctagctacagaagcgggcaaaggcccaacatgcgcgcttagtctatctcccgggaggggtcaggacacggaggc

SEQ ID NO: 340 - DNA, 28 bp, synthetic construct
  source 1..28: mol_type = other DNA
ctctggctccatcgtaagcaaaccttag

SEQ ID NO: 341 - DNA, 26 bp, synthetic construct
  source 1..26: mol_type = other DNA
cctccaacccgggcccctatgtccac

SEQ ID NO: 342 - DNA, 26 bp, synthetic construct
  source 1..26: mol_type = other DNA
cagacgcccagagaagggaagacacc

SEQ ID NO: 343 - DNA, 28 bp, synthetic construct
  source 1..28: mol_type = other DNA
ccgcgcctggtcacattgactttaattc

SEQ ID NO: 344 - DNA, 27 bp, synthetic construct
  source 1..27: mol_type = other DNA
gaagcgaggcatgaggatcacttgagg

SEQ ID NO: 345 - DNA, 27 bp, synthetic construct
  source 1..27: mol_type = other DNA
cctgacaaagctcagctcctctcctag

SEQ ID NO: 346 - DNA, 28 bp, synthetic construct
  source 1..28: mol_type = other DNA
gtgagatggctgaaaagcgatacagggc

SEQ ID NO: 347 - DNA, 27 bp, synthetic construct
  source 1..27: mol_type = other DNA
gccaccgatggagaggtctgccagtcc

SEQ ID NO: 348 - DNA, 26 bp, synthetic construct
  source 1..26: mol_type = other DNA
cttggttggtcaggcactgaagctcc

SEQ ID NO: 349 - DNA, 27 bp, synthetic construct
  source 1..27: mol_type = other DNA
ggatgtcatggagtggtgactgtggcc

SEQ ID NO: 350 - DNA, 27 bp, synthetic construct
  source 1..27: mol_type = other DNA
tcctgcagggagcttggcatgagaaac

SEQ ID NO: 351 - DNA, 27 bp, synthetic construct
  source 1..27: mol_type = other DNA
tgtcaaccagtatcccggtgcaggagc

SEQ ID NO: 352 - DNA, 28 bp, synthetic construct
  source 1..28: mol_type = other DNA
ccacgtattgcactgccattctaccaac

SEQ ID NO: 353 - DNA, 27 bp, synthetic construct
  source 1..27: mol_type = other DNA
gtccagccccatctgtcaaactgtgcg

SEQ ID NO: 354 - DNA, 30 bp, synthetic construct
  source 1..30: mol_type = other DNA
aattcttacatgcaggaacactcagcagac

SEQ ID NO: 355 - DNA, 27 bp, synthetic construct
  source 1..27: mol_type = other DNA
cacgccaacacagtttgctcacatgcc

SEQ ID NO: 356 - DNA, 27 bp, synthetic construct
  source 1..27: mol_type = other DNA
gggatagcacctcaaatgccagggagg

SEQ ID NO: 357 - DNA, 27 bp, synthetic construct
  source 1..27: mol_type = other DNA
atggcacgatacacacagacactgcag

SEQ ID NO: 358 - DNA, 26 bp, synthetic construct
  source 1..26: mol_type = other DNA
ggctggagcactgtctgcgcacaccg

SEQ ID NO: 359 - DNA, 26 bp, synthetic construct
  source 1..26: mol_type = other DNA
gcggcggcgagccgcgggcaggggcc

SEQ ID NO: 360 - DNA, 68 bp, synthetic construct
  source 1..68: mol_type = other DNA
tctccagccctggcctgggtcaatccttggggcccagactgagcacgtgatggcagaggaaaggaagc

SEQ ID NO: 361 - DNA, 68 bp, synthetic construct
  source 1..68: mol_type = other DNA
acttctcgcggctccgctcggctcggcttcccccgcgcggaccacggctcctccgaagcgagaacagc

SEQ ID NO: 362 - DNA, 65 bp, synthetic construct
  source 1..65: mol_type = other DNA
attgcttattgctgaggggcaaagtgaagaccaaggatagactgctgggcttgacagcatggagg

SEQ ID NO: 363 - DNA, 65 bp, synthetic construct
  source 1..65: mol_type = other DNA
agtctagtgcaagctaacagttgcttttatcacaggctccaggaagggtttggcctctgattagg

SEQ ID NO: 364 - DNA, 66 bp, synthetic construct
  source 1..66: mol_type = other DNA
agtacccagaaccagagccacattaaccggccctgggaatataaggtggtcccagctcggggacac

SEQ ID NO: 365 - DNA, 67 bp, synthetic construct
  source 1..67: mol_type = other DNA
ggtacagaagcgggcaaaggggcgaccggacccgagcccagggaggcgtacatagggggcgccgagg

SEQ ID NO: 366 - DNA, 66 bp, synthetic construct
  source 1..66: mol_type = other DNA
gatggtattcttcagactatagaaggagcttccagttgaattcaccagtggacaaaatgaggaaaa

SEQ ID NO: 367 - DNA, 65 bp, synthetic construct
  source 1..65: mol_type = other DNA
ggtgggtgggagtggcactttcactaggcctccgtatcactctctgactggggtatctcccagca

SEQ ID NO: 368 - DNA, 64 bp, synthetic construct
  source 1..64: mol_type = other DNA
tctgttttgtctgagggtgagggatgagataatgatgagtcagggcttcagggaaatgaacatt

SEQ ID NO: 369 - DNA, 65 bp, synthetic construct
  source 1..65: mol_type = other DNA
tttccagcccgctggccctgtaaaggaaactggaacacaaagcatagactgcggggcgggccagc

SEQ ID NO: 370 - DNA, 66 bp, synthetic construct
  source 1..66: mol_type = other DNA
gttcccatcaccatcaccaccaccaccaccatcaccaccaccatggacaacaagccttgggtaacc